European Patent Application EP 4 703 475 A1, published March 4, 2026. Title: NUCLEIC ACID ENCODING ANTI-VEGF PROTEIN, POLYNUCLEOTIDE EXPRESSION CASSETTE AND RECOMBINANT ADENO-ASSOCIATED VIRUS. Applicant: CHENGDU ORIGEN BIOTECHNOLOGY CO LTD. The sequence listing filed with the application follows.

SEQUENCE LISTING (34 sequences)

SEQ ID NO: 1 - protein, 432 aa, synthetic construct
SDTGRPFVEMYSEIPEIIHMTEGRELVIPCRVTSPNITVTLKKFPLDTLIPDGKRIIWDSRKGFIISNATYKEIGLLTCEATVNGHLYKTNYLTHRQTNTIIDVVLSPSHGIELSVGEKLVLNCTARTELNVGIDFNWEYPSSKHQHKKLVNRDLKTQSGSEMKKFLSTLTIDGVTRSDQGLYTCAASSGLMTKKNSTFVRVHEKDKTHTCPPCPAPELLGGPSVFLFPPKPKDTLMISRTPEVTCVVVDVSHEDPEVKFNWYVDGVEVHNAKTKPREEQYNSTYRVVSVLTVLHQDWLNGKEYKCKVSNKALPAPIEKTISKAKGQPREPQVYTLPPSRDELTKNQVSLTCLVKGFYPSDIAVEWESNGQPENNYKTTPPVLDSDGSFFLYSKLTVDKSRWQQGNVFSCSVMHEALHNHYTQKSLSLSPGK

SEQ ID NO: 2 - protein, 526 aa, synthetic construct
GRPFVEMYSEIPEIIHMTEGRELVIPCRVTSPNITVTLKKFPLDTLIPDGKRIIWDSRKGFIISNATYKEIGLLTCEATVNGHLYKTNYLTHRQTNTIIDVVLSPSHGIELSVGEKLVLNCTARTELNVGIDFNWEYPSSKHQHKKLVNRDLKTQSGSEMKKFLSTLTIDGVTRSDQGLYTCAASSGLMTKKNSTFVRVHEKPFVAFGSGMESLVEATVGERVRIPAKYLGYPPPEIKWYKNGIPLESNHTIKAGHVLTIMEVSERDTGNYTVILTNPISKEKQSHVVSLVVYVPPGPGDKTHTCPLCPAPELLGGPSVFLFPPKPKDTLMISRTPEVTCVVVDVSHEDPEVKFNWYVDGVEVHNAKTKPREEQYNSTYRVVSVLTVLHQDWLNGKEYKCKVSNKALPAPIEKTISKAKGQPREPQVYTLPPSRDELTKNQVSLTCLVKGFYPSDIAVEWESNGQPENNYKATPPVLDSDGSFFLYSKLTVDKSRWQQGNVFSCSVMHEALHNHYTQKSLSLSPGK

SEQ ID NO: 3 - DNA, 82 bp, synthetic construct
  source 1..82: mol_type = other DNA
gtgagtatctcagggatccagacatggggatatgggaggtgcctctgatcccagggctcactgtgggtctctctgttcacag

SEQ ID NO: 4 - DNA, 97 bp, synthetic construct
  source 1..97: mol_type = other DNA
gtaagtttagtctttttgtcttttatttcaggtcccggatccggtggtggtgcaaatcaaagaactgctcctcagtggatgttgcctttacttctag

SEQ ID NO: 5 - DNA, 60 bp, synthetic construct
  source 1..60: mol_type = other DNA
gtaagtatcaaggttacaagacaggtttaaggagaccaatagaaactgggcttgtcgaga

SEQ ID NO: 6 - DNA, 1459 bp, synthetic construct
  source 1..1459: mol_type = other DNA
atggtgtcctattgggatacaggagtgctgctgtgtgctctgctgagctgtctgctgctgacaggctcttcttcaggcaggtgagtatctcagggatccagacatggggatatgggaggtgcctctgatcccagggctcactgtgggtctctctgttcacagggacacaggcagaccctttgtggagatgtactctgaaatccctgagatcattcacatgacagaaggcagagaactggtgattccctgcagggttaccagcccaaacatcacagtgaccctgaagaagttccccctggacaccctgatccctgatggcaaaagaatcatctgggactctaggaaaggctttatcatctccaatgccacatacaaagagattggcctgctgacctgtgaggctactgtcaatggccacctgtacaaaacaaattacctgacccacagacagaccaacacaatcattgatgtggtgctgagcccatcccatggcattgagctgtctgtgggagaaaagctggtgctgaattgtacagctagaacagaacttaatgtgggcattgatttcaactgggagtaccctagctccaagcaccagcataaaaagctggtgaacagagacctgaagacccagtctggctctgagatgaaaaagttcttgagcaccctgaccattgatggagtgaccagatctgaccagggcctgtacacctgtgctgcctcctctgggctgatgacaaaaaagaacagcacctttgtgagagtgcatgagaaggataaaacccacacctgccctccttgtcctgctcctgagctgctggggggaccatctgtgttcctgttcccccccaagcccaaggataccctgatgatcagcagaaccccagaagtgacctgtgtggtggtggatgtgtcccatgaggacccagaggtgaaattcaactggtatgtggatggagtggaggtgcacaatgccaagaccaaaccaagagaggagcagtataactccacctacagggtggtgtctgtgctgactgtgctgcaccaggattggctgaatggcaaggagtacaagtgcaaggttagcaataaagctctgcctgcccccattgaaaagaccatttccaaagccaaagggcagccaagggagccccaggtgtacaccctgcccccatctagagatgagctgaccaagaaccaggtgagcctcacatgtctggtgaagggcttttacccttctgacattgctgtggagtgggaaagcaatggacagcctgagaataactataagaccacacccccagtgctggattctgatggcagttttttcctgtactctaagctgacagtggacaaatccagatggcagcagggcaatgtgttcagctgctctgtgatgcatgaggccctgcacaatcactatacacagaagagcctgagcctgagcccagggaagtga

SEQ ID NO: 7 - DNA, 1377 bp, synthetic construct
  source 1..1377: mol_type = other DNA
atggtgtcctattgggatacaggagtgctgctgtgtgctctgctgagctgtctgctgctgacaggctcttcttcaggcagcgacaccggccggcccttcgtggagatgtacagcgaaatccctgagatcattcacatgacagaaggccgcgaactggtgattccctgcagggttaccagcccaaacatcaccgtgaccctgaagaagttccccctggacaccctgatccctgacggcaaacggatcatctgggactctaggaaaggctttatcatctccaatgccacatacaaagagattggcctgctgacctgcgaggctacggtcaacggccacctgtacaaaacaaattacctgacccacagacagaccaacacaatcatcgacgtggtgctgagcccatcccatggcattgagctgtccgtgggagaaaagctggtgctgaattgtacggctagaacagaacttaacgtgggcatcgatttcaactgggagtaccctagctccaagcaccagcataaaaagctggtgaaccgggacctgaagacccagtccggcagtgagatgaaaaagttcttgagcaccctgaccatcgatggagtgacccgaagcgaccagggcctgtacacctgtgccgcctcctctgggctgatgacaaaaaagaacagcacctttgtcagagtgcacgagaaggataaaacccacacctgccctccttgtcccgctcctgagctgctggggggaccatctgtgttcctgttcccccccaagcccaaggataccctgatgatcagccgaaccccagaagtgacctgcgtggtggtggacgtgtcccacgaggacccagaggtgaaattcaactggtatgtggacggcgtggaggtgcacaatgccaagaccaaaccaagagaggagcagtataactccacctacagggtggtgagcgtgctgactgtgctgcaccaggattggctgaacggcaaggagtacaagtgcaaggttagcaataaagctctgcccgcccccatcgaaaagaccatttccaaagccaaagggcagccaagggagccccaggtgtacaccctgcccccatctcgggacgagctgaccaagaaccaggtgagtctcacatgtctcgtgaagggcttttaccctagcgacatcgccgtcgagtgggaaagcaacggacagcctgagaataactataagaccacaccccccgtgctggattccgacggcagttttttcctgtactctaagctgacagtggacaaatcccgctggcagcagggcaacgtgttcagctgctccgtgatgcacgaggccctgcacaatcactatacacagaagagcctgagcctgagccccgggaagtga

SEQ ID NO: 8 - DNA, 1377 bp, synthetic construct
  source 1..1377: mol_type = other DNA
atggtgtcctattgggatacaggagtgctgctgtgtgctctgctgagctgtctgctgctgacaggctcttcttcaggctctgacacaggcagaccctttgtggagatgtactctgaaatccctgagatcattcacatgacagaaggcagagaactggtgattccctgcagggttaccagcccaaacatcacagtgaccctgaagaagttccccctggacaccctgatccctgatggcaaaagaatcatctgggactctaggaaaggctttatcatctccaatgccacatacaaagagattggcctgctgacctgtgaggctactgtcaatggccacctgtacaaaacaaattacctgacccacagacagaccaacacaatcattgatgtggtgctgagcccatcccatggcattgagctgtctgtgggagaaaagctggtgctgaattgtacagctagaacagaacttaatgtgggcattgatttcaactgggagtaccctagctccaagcaccagcataaaaagctggtgaacagagacctgaagacccagtctggctctgagatgaaaaagttcttgagcaccctgaccattgatggagtgaccagatctgaccagggcctgtacacctgtgctgcctcctctgggctgatgacaaaaaagaacagcacctttgtgagagtgcatgagaaggataaaacccacacctgccctccttgtcctgctcctgagctgctggggggaccatctgtgttcctgttcccccccaagcccaaggataccctgatgatcagcagaaccccagaagtgacctgtgtggtggtggatgtgtcccatgaggacccagaggtgaaattcaactggtatgtggatggagtggaggtgcacaatgccaagaccaaaccaagagaggagcagtataactccacctacagggtggtgtctgtgctgactgtgctgcaccaggattggctgaatggcaaggagtacaagtgcaaggttagcaataaagctctgcctgcccccattgaaaagaccatttccaaagccaaagggcagccaagggagccccaggtgtacaccctgcccccatctagagatgagctgaccaagaaccaggtgagcctcacatgtctggtgaagggcttttacccttctgacattgctgtggagtgggaaagcaatggacagcctgagaataactataagaccacacccccagtgctggattctgatggcagttttttcctgtactctaagctgacagtggacaaatccagatggcagcagggcaatgtgttcagctgctctgtgatgcatgaggccctgcacaatcactatacacagaagagcctgagcctgagcccagggaagtga

SEQ ID NO: 9 - DNA, 3781 bp, synthetic construct
  source 1..3781: mol_type = other DNA
ctgcgcgctcgctcgctcactgaggccgcccgggcaaagcccgggcgtcgggcgacctttggtcgcccggcctcagtgagcgagcgagcgcgcagagagggagtggccaactccatcactaggggttccttgtagttaatgattaacccgccatgctacttatctaccagggtaatggggatcctctagaactatagctagtcgacattgattattgactagttattaatagtaatcaattacggggtcattagttcatagcccatatatggagttccgcgttacataacttacggtaaatggcccgcctggctgaccgcccaacgacccccgcccattgacgtcaataatgacgtatgttcccatagtaacgccaatagggactttccattgacgtcaatgggtggagtatttacggtaaactgcccacttggcagtacatcaagtgtatcatatgccaagtacgccccctattgacgtcaatgacggtaaatggcccgcctggcattatgcccagtacatgaccttatgggactttcctacttggcagtacatctacgtattagtcatcgctattaccatggtcgaggtgagccccacgttctgcttcactctccccatctcccccccctccccacccccaattttgtatttatttattttttaattattttgtgcagcgatgggggcggggggggggggggggcgcgcgccaggcggggcggggcggggcgaggggcggggcggggcgaggcggagaggtgcggcggcagccaatcagagcggcgcgctccgaaagtttccttttatggcgaggcggcggcggcggcggccctataaaaagcgaagcgcgcggcgggcggggagtcgctgcgacgctgccttcgccccgtgccccgctccgccgccgcctcgcgccgcccgccccggctctgactgaccgcgttactcccacaggtgagcgggcgggacggcccttctcctccgggctgtaattagcgcttggtttaatgacggcttgtttcttttctgtggctgcgtgaaagccttgaggggctccgggagggccctttgtgcggggggagcggctcggggggtgcgtgcgtgtgtgtgtgcgtggggagcgccgcgtgcggctccgcgctgcccggcggctgtgagcgctgcgggcgcggcgcggggctttgtgcgctccgcagtgtgcgcgaggggagcgcggccgggggcggtgccccgcggtgcggggggggctgcgaggggaacaaaggctgcgtgcggggtgtgtgcgtgggggggtgagcagggggtgtgggcgcgtcggtcgggctgcaaccccccctgcacccccctccccgagttgctgagcacggcccggcttcgggtgcggggctccgtacggggcgtggcgcggggctcgccgtgccgggcggggggtggcggcaggtgggggtgccgggcggggcggggccgcctcgggccggggagggctcgggggaggggcgcggcggcccccggagcgccggcggctgtcgaggcgcggcgagccgcagccattgccttttatggtaatcgtgcgagagggcgcagggacttcctttgtcccaaatctgtgcggagccgaaatctgggaggcgccgccgcaccccctctagcgggcgcggggcgaagcggtgcggcgccggcaggaaggaaatgggcggggagggccttcgtgcgtcgccgcgccgccgtccccttctccctctccagcctcggggctgtccgcggggggacggctgccttcgggggggacggggcagggcggggttcggcttctggcgtgtgaccggcggctctagagcctctgctaaccatgttcatgccttcttctttttcctacagctcctgggcaacgtgctggttattgtgctgtctcatcattttggcaaagaattcgccgccaccatggtgtcctattgggatacaggagtgctgctgtgtgctctgctgagctgtctgctgctgacaggctcttcttcaggcaggtgagtatctcagggatccagacatggggatatgggaggtgcctctgatcccagggctcactgtgggtctctctgttcacagggacacaggcagaccctttgtggagatgtactctgaaatccctgagatcattcacatgacagaaggcagagaactggtgattccctgcagggttaccagcccaaacatcacagtgaccctgaagaagttccccctggacaccctgatccctgatggcaaaagaatcatctgggactctaggaaaggctttatcatctccaatgccacatacaaagagattggcctgctgacctgtgaggctactgtcaatggccacctgtacaaaacaaattacctgacccacagacagaccaacacaatcattgatgtggtgctgagcccatcccatggcattgagctgtctgtgggagaaaagctggtgctgaattgtacagctagaacagaacttaatgtgggcattgatttcaactgggagtaccctagctccaagcaccagcataaaaagctggtgaacagagacctgaagacccagtctggctctgagatgaaaaagttcttgagcaccctgaccattgatggagtgaccagatctgaccagggcctgtacacctgtgctgcctcctctgggctgatgacaaaaaagaacagcacctttgtgagagtgcatgagaaggataaaacccacacctgccctccttgtcctgctcctgagctgctggggggaccatctgtgttcctgttcccccccaagcccaaggataccctgatgatcagcagaaccccagaagtgacctgtgtggtggtggatgtgtcccatgaggacccagaggtgaaattcaactggtatgtggatggagtggaggtgcacaatgccaagaccaaaccaagagaggagcagtataactccacctacagggtggtgtctgtgctgactgtgctgcaccaggattggctgaatggcaaggagtacaagtgcaaggttagcaataaagctctgcctgcccccattgaaaagaccatttccaaagccaaagggcagccaagggagccccaggtgtacaccctgcccccatctagagatgagctgaccaagaaccaggtgagcctcacatgtctggtgaagggcttttacccttctgacattgctgtggagtgggaaagcaatggacagcctgagaataactataagaccacacccccagtgctggattctgatggcagttttttcctgtactctaagctgacagtggacaaatccagatggcagcagggcaatgtgttcagctgctctgtgatgcatgaggccctgcacaatcactatacacagaagagcctgagcctgagcccagggaagtgactcgaggacggggtgaactacgcctgaggatccgatctttttccctctgccaaaaattatggggacatcatgaagccccttgagcatctgacttctggctaataaaggaaatttattttcattgcaatagtgtgttggaattttttgtgtctctcactcggaagcaattcgttgatctgaatttcgaccacccataatacccattaccctggtagataagtagcatggcgggttaatcattaactacaaggaacccctagtgatggagttggccactccctctctgcgcgctcgctcgctcactgaggccgggcgaccaaaggtcgcccgacgcccgggctttgcccgggcggcctcagtgagcgagcgagcgcgcag

SEQ ID NO: 10 - DNA, 6536 bp, synthetic construct
  source 1..6536: mol_type = other DNA
ctcgaggacggggtgaactacgcctgaggatccgatctttttccctctgccaaaaattatggggacatcatgaagccccttgagcatctgacttctggctaataaaggaaatttattttcattgcaatagtgtgttggaattttttgtgtctctcactcggaagcaattcgttgatctgaatttcgaccacccataatacccattaccctggtagataagtagcatggcgggttaatcattaactacaaggaacccctagtgatggagttggccactccctctctgcgcgctcgctcgctcactgaggccgggcgaccaaaggtcgcccgacgcccgggctttgcccgggcggcctcagtgagcgagcgagcgcgcagccttaattaacctaattcactggccgtcgttttacaacgtcgtgactgggaaaaccctggcgttacccaacttaatcgccttgcagcacatccccctttcgccagctggcgtaatagcgaagaggcccgcaccgatcgcccttcccaacagttgcgcagcctgaatggcgaatgggacgcgccctgtagcggcgcattaagcgcggcgggtgtggtggttacgcgcagcgtgaccgctacacttgccagcgccctagcgcccgctcctttcgctttcttcccttcctttctcgccacgttcgccggctttccccgtcaagctctaaatcgggggctccctttagggttccgatttagtgctttacggcacctcgaccccaaaaaacttgattagggtgatggttcacgtagtgggccatcgccctgatagacggtttttcgccctttgacgttggagtccacgttctttaatagtggactcttgttccaaactggaacaacactcaaccctatctcggtctattcttttgatttataagggattttgccgatttcggcctattggttaaaaaatgagctgatttaacaaaaatttaacgcgaattttaacaaaatattaacgcttacaatttaggtggcacttttcggggaaatgtgcgcggaacccctatttgtttatttttctaaatacattcaaatatgtatccgctcatgagacaataaccctgataaatgcttcaataatattgaaaaaggaagagtatgattgaacaagatggattgcacgcaggttctccggccgcttgggtggagaggctattcggctatgactgggcacaacagacaatcggctgctctgatgccgccgtgttccggctgtcagcgcaggggcgcccggttctttttgtcaagaccgacctgtccggtgccctgaatgaactgcaagacgaggcagcgcggctatcgtggctggccacgacgggcgttccttgcgcagctgtgctcgacgttgtcactgaagcgggaagggactggctgctattgggcgaagtgccggggcaggatctcctgtcatctcaccttgctcctgccgagaaagtatccatcatggctgatgcaatgcggcggctgcatacgcttgatccggctacctgcccattcgaccaccaagcgaaacatcgcatcgagcgagcacgtactcggatggaagccggtcttgtcgatcaggatgatctggacgaagagcatcaggggctcgcgccagccgaactgttcgccaggctcaaggcgagcatgcccgacggcgaggatctcgtcgtgacccatggcgatgcctgcttgccgaatatcatggtggaaaatggccgcttttctggattcatcgactgtggccggctgggtgtggcggaccgctatcaggacatagcgttggctacccgtgatattgctgaagagcttggcggcgaatgggctgaccgcttcctcgtgctttacggtatcgccgctcccgattcgcagcgcatcgccttctatcgccttcttgacgagttcttctgactgtcagaccaagtttactcatatatactttagattgatttaaaacttcatttttaatttaaaaggatctaggtgaagatcctttttgataatctcatgaccaaaatcccttaacgtgagttttcgttccactgagcgtcagaccccgtagaaaagatcaaaggatcttcttgagatcctttttttctgcgcgtaatctgctgcttgcaaacaaaaaaaccaccgctaccagcggtggtttgtttgccggatcaagagctaccaactctttttccgaaggtaactggcttcagcagagcgcagataccaaatactgttcttctagtgtagccgtagttaggccaccacttcaagaactctgtagcaccgcctacatacctcgctctgctaatcctgttaccagtggctgctgccagtggcgataagtcgtgtcttaccgggttggactcaagacgatagttaccggataaggcgcagcggtcgggctgaacggggggttcgtgcacacagcccagcttggagcgaacgacctacaccgaactgagatacctacagcgtgagctatgagaaagcgccacgcttcccgaagggagaaaggcggacaggtatccggtaagcggcagggtcggaacaggagagcgcacgagggagcttccagggggaaacgcctggtatctttatagtcctgtcgggtttcgccacctctgacttgagcgtcgatttttgtgatgctcgtcaggggggcggagcctatggaaaaacgccagcaacgcggcctttttacggttcctggccttttgctggccttttgctcacatgttctttcctgcgttatcccctgattctgtggataaccgtattaccgcctttgagtgagctgataccgctcgccgcagccgaacgaccgagcgcagcgagtcagtgagcgaggaagcggaagagcgcccaatacgcaaaccgcctctccccgcgcgttggccgattcattaatgcagctggcacgacaggtttcccgactggaaagcgggcagtgagcgcaacgcaattaatgtgagttagctcactcattaggcaccccaggctttacactttatgcttccggctcgtatgttgtgtggaattgtgagcggataacaatttcacacaggaaacagctatgaccatgattacgccagatttaattaaggccttaattaggctgcgcgctcgctcgctcactgaggccgcccgggcaaagcccgggcgtcgggcgacctttggtcgcccggcctcagtgagcgagcgagcgcgcagagagggagtggccaactccatcactaggggttccttgtagttaatgattaacccgccatgctacttatctaccagggtaatggggatcctctagaactatagctagtcgacattgattattgactagttattaatagtaatcaattacggggtcattagttcatagcccatatatggagttccgcgttacataacttacggtaaatggcccgcctggctgaccgcccaacgacccccgcccattgacgtcaataatgacgtatgttcccatagtaacgccaatagggactttccattgacgtcaatgggtggagtatttacggtaaactgcccacttggcagtacatcaagtgtatcatatgccaagtacgccccctattgacgtcaatgacggtaaatggcccgcctggcattatgcccagtacatgaccttatgggactttcctacttggcagtacatctacgtattagtcatcgctattaccatggtcgaggtgagccccacgttctgcttcactctccccatctcccccccctccccacccccaattttgtatttatttattttttaattattttgtgcagcgatgggggcggggggggggggggggcgcgcgccaggcggggcggggcggggcgaggggcggggcggggcgaggcggagaggtgcggcggcagccaatcagagcggcgcgctccgaaagtttccttttatggcgaggcggcggcggcggcggccctataaaaagcgaagcgcgcggcgggcggggagtcgctgcgacgctgccttcgccccgtgccccgctccgccgccgcctcgcgccgcccgccccggctctgactgaccgcgttactcccacaggtgagcgggcgggacggcccttctcctccgggctgtaattagcgcttggtttaatgacggcttgtttcttttctgtggctgcgtgaaagccttgaggggctccgggagggccctttgtgcggggggagcggctcggggggtgcgtgcgtgtgtgtgtgcgtggggagcgccgcgtgcggctccgcgctgcccggcggctgtgagcgctgcgggcgcggcgcggggctttgtgcgctccgcagtgtgcgcgaggggagcgcggccgggggcggtgccccgcggtgcggggggggctgcgaggggaacaaaggctgcgtgcggggtgtgtgcgtgggggggtgagcagggggtgtgggcgcgtcggtcgggctgcaaccccccctgcacccccctccccgagttgctgagcacggcccggcttcgggtgcggggctccgtacggggcgtggcgcggggctcgccgtgccgggcggggggtggcggcaggtgggggtgccgggcggggcggggccgcctcgggccggggagggctcgggggaggggcgcggcggcccccggagcgccggcggctgtcgaggcgcggcgagccgcagccattgccttttatggtaatcgtgcgagagggcgcagggacttcctttgtcccaaatctgtgcggagccgaaatctgggaggcgccgccgcaccccctctagcgggcgcggggcgaagcggtgcggcgccggcaggaaggaaatgggcggggagggccttcgtgcgtcgccgcgccgccgtccccttctccctctccagcctcggggctgtccgcggggggacggctgccttcgggggggacggggcagggcggggttcggcttctggcgtgtgaccggcggctctagagcctctgctaaccatgttcatgccttcttctttttcctacagctcctgggcaacgtgctggttattgtgctgtctcatcattttggcaaagaattcgccgccaccatggtgtcctattgggatacaggagtgctgctgtgtgctctgctgagctgtctgctgctgacaggctcttcttcaggcaggtgagtatctcagggatccagacatggggatatgggaggtgcctctgatcccagggctcactgtgggtctctctgttcacagggacacaggcagaccctttgtggagatgtactctgaaatccctgagatcattcacatgacagaaggcagagaactggtgattccctgcagggttaccagcccaaacatcacagtgaccctgaagaagttccccctggacaccctgatccctgatggcaaaagaatcatctgggactctaggaaaggctttatcatctccaatgccacatacaaagagattggcctgctgacctgtgaggctactgtcaatggccacctgtacaaaacaaattacctgacccacagacagaccaacacaatcattgatgtggtgctgagcccatcccatggcattgagctgtctgtgggagaaaagctggtgctgaattgtacagctagaacagaacttaatgtgggcattgatttcaactgggagtaccctagctccaagcaccagcataaaaagctggtgaacagagacctgaagacccagtctggctctgagatgaaaaagttcttgagcaccctgaccattgatggagtgaccagatctgaccagggcctgtacacctgtgctgcctcctctgggctgatgacaaaaaagaacagcacctttgtgagagtgcatgagaaggataaaacccacacctgccctccttgtcctgctcctgagctgctggggggaccatctgtgttcctgttcccccccaagcccaaggataccctgatgatcagcagaaccccagaagtgacctgtgtggtggtggatgtgtcccatgaggacccagaggtgaaattcaactggtatgtggatggagtggaggtgcacaatgccaagaccaaaccaagagaggagcagtataactccacctacagggtggtgtctgtgctgactgtgctgcaccaggattggctgaatggcaaggagtacaagtgcaaggttagcaataaagctctgcctgcccccattgaaaagaccatttccaaagccaaagggcagccaagggagccccaggtgtacaccctgcccccatctagagatgagctgaccaagaaccaggtgagcctcacatgtctggtgaagggcttttacccttctgacattgctgtggagtgggaaagcaatggacagcctgagaataactataagaccacacccccagtgctggattctgatggcagttttttcctgtactctaagctgacagtggacaaatccagatggcagcagggcaatgtgttcagctgctctgtgatgcatgaggccctgcacaatcactatacacagaagagcctgagcctgagcccagggaagtga

SEQ ID NO: 11 - protein, 10 aa, synthetic construct
RGNQQNTARQ

SEQ ID NO: 12 - DNA, 1359 bp, synthetic construct
  source 1..1359: mol_type = other DNA
atgtacagaatgcagctgctgctgctgatcgccctgagcctggccctggtgaccaacagcagcgacaccggtagacctttcgtagagatgtacagtgaaatccccgaaattatacacatgactgaaggaagggagctcgtcattccctgccgggttacgtcacctaacatcactgttactttaaaaaagtttccacttgacactttgatccctgatggaaaacgcataatctgggacagtagaaagggcttcatcatatcaaatgcaacgtacaaagaaatagggcttctgacctgtgaagcaacagtcaatgggcatttgtataagacaaactatctcacacatcgacaaaccaatacaatcatagatgtggttctgagtccgtctcatggaattgaactatctgttggagaaaagcttgtcttaaattgtacagcaagaactgaactaaatgtggggattgacttcaactgggaatacccttcttcgaagcatcagcataagaaacttgtaaaccgagacctaaaaacccagtctgggagtgagatgaagaaatttttgagcaccttaactatagatggtgtaacccggagtgaccaaggattgtacacctgtgcagcatccagtgggctgatgaccaagaagaacagcacatttgtcagggtccatgaaaaagacaaaactcacacatgcccaccgtgcccagcacctgaactcctggggggaccgtcagtcttcctcttccccccaaaacccaaggacaccctcatgatctcccggacccctgaggtcacatgcgtggtggtggacgtgagccacgaagaccctgaggtcaagttcaactggtacgtggacggcgtggaggtgcataatgccaagacaaagccgcgggaggagcagtacaacagcacgtaccgtgtggtcagcgtcctcaccgtcctgcaccaggactggctgaatggcaaggagtacaagtgcaaggtctccaacaaagccctcccagcccccatcgagaaaaccatctccaaagccaaagggcagccccgagaaccacaggtgtacaccctgcccccatcccgggatgagctgaccaagaaccaggtcagcctgacctgcctggtcaaaggcttctatcccagcgacatcgccgtggagtgggagagcaatgggcagccggagaacaactacaagaccacgcctcccgtgctggactccgacggctccttcttcctctatagcaagctcaccgtggacaagagcaggtggcagcaggggaacgtcttctcatgctccgtgatgcatgaggctctgcacaaccactacacgcagaagagcctctccctgtctccgggtaaataa

SEQ ID NO: 13 - DNA, 1459 bp, synthetic construct
  source 1..1459: mol_type = other DNA
atggtgtcctattgggatacaggagtgctgctgtgtgctctgctgagctgtctgctgctgacaggctcttcttcaggctctgacacaggcagaccctttgtggagatgtactctgaaatccctgagatcattcacatgacagaaggcagagaactggtgattccctgcagggttaccagcccaaacatcacagtgaccctgaagaagttccccctggacaccctgatccctgatggcaaaagaatcatctgggactctaggtgagtatctcagggatccagacatggggatatgggaggtgcctctgatcccagggctcactgtgggtctctctgttcacaggaaaggctttatcatctccaatgccacatacaaagagattggcctgctgacctgtgaggctactgtcaatggccacctgtacaaaacaaattacctgacccacagacagaccaacacaatcattgatgtggtgctgagcccatcccatggcattgagctgtctgtgggagaaaagctggtgctgaattgtacagctagaacagaacttaatgtgggcattgatttcaactgggagtaccctagctccaagcaccagcataaaaagctggtgaacagagacctgaagacccagtctggctctgagatgaaaaagttcttgagcaccctgaccattgatggagtgaccagatctgaccagggcctgtacacctgtgctgcctcctctgggctgatgacaaaaaagaacagcacctttgtgagagtgcatgagaaggataaaacccacacctgccctccttgtcctgctcctgagctgctggggggaccatctgtgttcctgttcccccccaagcccaaggataccctgatgatcagcagaaccccagaagtgacctgtgtggtggtggatgtgtcccatgaggacccagaggtgaaattcaactggtatgtggatggagtggaggtgcacaatgccaagaccaaaccaagagaggagcagtataactccacctacagggtggtgtctgtgctgactgtgctgcaccaggattggctgaatggcaaggagtacaagtgcaaggttagcaataaagctctgcctgcccccattgaaaagaccatttccaaagccaaagggcagccaagggagccccaggtgtacaccctgcccccatctagagatgagctgaccaagaaccaggtgagcctcacatgtctggtgaagggcttttacccttctgacattgctgtggagtgggaaagcaatggacagcctgagaataactataagaccacacccccagtgctggattctgatggcagttttttcctgtactctaagctgacagtggacaaatccagatggcagcagggcaatgtgttcagctgctctgtgatgcatgaggccctgcacaatcactatacacagaagagcctgagcctgagcccagggaagtga

SEQ ID NO: 14 - DNA, 130 bp, synthetic construct
  source 1..130: mol_type = other DNA
ctgcgcgctcgctcgctcactgaggccgcccgggcaaagcccgggcgtcgggcgacctttggtcgcccggcctcagtgagcgagcgagcgcgcagagagggagtggccaactccatcactaggggttcct

SEQ ID NO: 15 - DNA, 666 bp, synthetic construct
  source 1..666: mol_type = other DNA
ctagtcgacattgattattgactagttattaatagtaatcaattacggggtcattagttcatagcccatatatggagttccgcgttacataacttacggtaaatggcccgcctggctgaccgcccaacgacccccgcccattgacgtcaataatgacgtatgttcccatagtaacgccaatagggactttccattgacgtcaatgggtggagtatttacggtaaactgcccacttggcagtacatcaagtgtatcatatgccaagtacgccccctattgacgtcaatgacggtaaatggcccgcctggcattatgcccagtacatgaccttatgggactttcctacttggcagtacatctacgtattagtcatcgctattaccatggtcgaggtgagccccacgttctgcttcactctccccatctcccccccctccccacccccaattttgtatttatttattttttaattattttgtgcagcgatgggggcggggggggggggggggcgcgcgccaggcggggcggggcggggcgaggggcggggcggggcgaggcggagaggtgcggcggcagccaatcagagcggcgcgctccgaaagtttccttttatggcgaggcggcggcggcggcggccctataaaaagcgaagcgcgcggcgggcgg

SEQ ID NO: 16 - DNA, 972 bp, synthetic construct
  source 1..972: mol_type = other DNA
gtgagcgggcgggacggcccttctcctccgggctgtaattagcgcttggtttaatgacggcttgtttcttttctgtggctgcgtgaaagccttgaggggctccgggagggccctttgtgcggggggagcggctcggggggtgcgtgcgtgtgtgtgtgcgtggggagcgccgcgtgcggctccgcgctgcccggcggctgtgagcgctgcgggcgcggcgcggggctttgtgcgctccgcagtgtgcgcgaggggagcgcggccgggggcggtgccccgcggtgcggggggggctgcgaggggaacaaaggctgcgtgcggggtgtgtgcgtgggggggtgagcagggggtgtgggcgcgtcggtcgggctgcaaccccccctgcacccccctccccgagttgctgagcacggcccggcttcgggtgcggggctccgtacggggcgtggcgcggggctcgccgtgccgggcggggggtggcggcaggtgggggtgccgggcggggcggggccgcctcgggccggggagggctcgggggaggggcgcggcggcccccggagcgccggcggctgtcgaggcgcggcgagccgcagccattgccttttatggtaatcgtgcgagagggcgcagggacttcctttgtcccaaatctgtgcggagccgaaatctgggaggcgccgccgcaccccctctagcgggcgcggggcgaagcggtgcggcgccggcaggaaggaaatgggcggggagggccttcgtgcgtcgccgcgccgccgtccccttctccctctccagcctcggggctgtccgcggggggacggctgccttcgggggggacggggcagggcggggttcggcttctggcgtgtgaccggcggctctagagcctctgctaaccatgttcatgccttcttctttttcctacagctcctgggcaacgtgctggttattgtgctgtctcatcattttggcaaa

SEQ ID NO: 17 - DNA, 13 bp, synthetic construct
  source 1..13: mol_type = other DNA
gccgccaccatgg

SEQ ID NO: 18 - DNA, 127 bp, synthetic construct
  source 1..127: mol_type = other DNA
gatctttttccctctgccaaaaattatggggacatcatgaagccccttgagcatctgacttctggctaataaaggaaatttattttcattgcaatagtgtgttggaattttttgtgtctctcactcg

SEQ ID NO: 19 - DNA, 130 bp, synthetic construct
  source 1..130: mol_type = other DNA
aggaacccctagtgatggagttggccactccctctctgcgcgctcgctcgctcactgaggccgggcgaccaaaggtcgcccgacgcccgggctttgcccgggcggcctcagtgagcgagcgagcgcgcag

SEQ ID NO: 20 - DNA, 133 bp, synthetic construct
  source 1..133: mol_type = other DNA
gtaagtatcaaggttacaagacaggtttaaggagaccaatagaaactgggcttgtcgagacagagaagactcttgcgtttctgataggcacctattggtcttactgacatccactttgcctttctctccacag

SEQ ID NO: 21 - DNA, 1474 bp, synthetic construct
  source 1..1474: mol_type = other DNA
atggtgtcctattgggatacaggagtgctgctgtgtgctctgctgagctgtctgctgctgacaggctcttcttcaggcaggtaagtttagtctttttgtcttttatttcaggtcccggatccggtggtggtgcaaatcaaagaactgctcctcagtggatgttgcctttacttctagggacacaggcagaccctttgtggagatgtactctgaaatccctgagatcattcacatgacagaaggcagagaactggtgattccctgcagggttaccagcccaaacatcacagtgaccctgaagaagttccccctggacaccctgatccctgatggcaaaagaatcatctgggactctaggaaaggctttatcatctccaatgccacatacaaagagattggcctgctgacctgtgaggctactgtcaatggccacctgtacaaaacaaattacctgacccacagacagaccaacacaatcattgatgtggtgctgagcccatcccatggcattgagctgtctgtgggagaaaagctggtgctgaattgtacagctagaacagaacttaatgtgggcattgatttcaactgggagtaccctagctccaagcaccagcataaaaagctggtgaacagagacctgaagacccagtctggctctgagatgaaaaagttcttgagcaccctgaccattgatggagtgaccagatctgaccagggcctgtacacctgtgctgcctcctctgggctgatgacaaaaaagaacagcacctttgtgagagtgcatgagaaggataaaacccacacctgccctccttgtcctgctcctgagctgctggggggaccatctgtgttcctgttcccccccaagcccaaggataccctgatgatcagcagaaccccagaagtgacctgtgtggtggtggatgtgtcccatgaggacccagaggtgaaattcaactggtatgtggatggagtggaggtgcacaatgccaagaccaaaccaagagaggagcagtataactccacctacagggtggtgtctgtgctgactgtgctgcaccaggattggctgaatggcaaggagtacaagtgcaaggttagcaataaagctctgcctgcccccattgaaaagaccatttccaaagccaaagggcagccaagggagccccaggtgtacaccctgcccccatctagagatgagctgaccaagaaccaggtgagcctcacatgtctggtgaagggcttttacccttctgacattgctgtggagtgggaaagcaatggacagcctgagaataactataagaccacacccccagtgctggattctgatggcagttttttcctgtactctaagctgacagtggacaaatccagatggcagcagggcaatgtgttcagctgctctgtgatgcatgaggccctgcacaatcactatacacagaagagcctgagcctgagcccagggaagtga

SEQ ID NO: 22 - DNA, 1459 bp, synthetic construct; identical to SEQ ID NO: 6
  source 1..1459: mol_type = other DNA

SEQ ID NO: 23 - DNA, 3794 bp, synthetic construct
  source 1..3794: mol_type = other DNA
ctgcgcgctcgctcgctcactgaggccgcccgggcaaagcccgggcgtcgggcgacctttggtcgcccggcctcagtgagcgagcgagcgcgcagagagggagtggccaactccatcactaggggttccttgtagttaatgattaacccgccatgctacttatctaccagggtaatggggatcctctagaactatagctagtcgacattgattattgactagttattaatagtaatcaattacggggtcattagttcatagcccatatatggagttccgcgttacataacttacggtaaatggcccgcctggctgaccgcccaacgacccccgcccattgacgtcaataatgacgtatgttcccatagtaacgccaatagggactttccattgacgtcaatgggtggagtatttacggtaaactgcccacttggcagtacatcaagtgtatcatatgccaagtacgccccctattgacgtcaatgacggtaaatggcccgcctggcattatgcccagtacatgaccttatgggactttcctacttggcagtacatctacgtattagtcatcgctattaccatggtcgaggtgagccccacgttctgcttcactctccccatctcccccccctccccacccccaattttgtatttatttattttttaattattttgtgcagcgatgggggcggggggggggggggggcgcgcgccaggcggggcggggcggggcgaggggcggggcggggcgaggcggagaggtgcggcggcagccaatcagagcggcgcgctccgaaagtttccttttatggcgaggcggcggcggcggcggccctataaaaagcgaagcgcgcggcgggcgggagtcgctgcgcgctgccttcgccccgtgccccgctccgccgccgcctcgcgccgcccgccccggctctgactgaccgcgttactcccacaggtgagcgggcgggacggcccttctcctccgggctgtaattagcgcttggtttaatgacggcttgtttcttttctgtggctgcgtgaaagccttgaggggctccgggagggccctttgtgcggggggagcggctcggggggtgcgtgcgtgtgtgtgtgcgtggggagcgccgcgtgcggctccgcgctgcccggcggctgtgagcgctgcgggcgcggcgcggggctttgtgcgctccgcagtgtgcgcgaggggagcgcggccgggggcggtgccccgcggtgcggggggggctgcgaggggaacaaaggctgcgtgcggggtgtgtgcgtgggggggtgagcagggggtgtgggcgcgtcggtcgggctgcaaccccccctgcacccccctccccgagttgctgagcacggcccggcttcgggtgcggggctccgtacggggcgtggcgcggggctcgccgtgccgggcggggggtggcggcaggtgggggtgccgggcggggcggggccgcctcgggccggggagggctcgggggaggggcgcggcggcccccggagcgccggcggctgtcgaggcgcggcgagccgcagccattgccttttatggtaatcgtgcgagagggcgcagggacttcctttgtcccaaatctgtgcggagccgaaatctgggaggcgccgccgcaccccctctagcgggcgcggggcgaagcggtgcggcgccggcaggaaggaaatgggcggggagggccttcgtgcgtcgccgcgccgccgtccccttctccctctccagcctcggggctgtccgcggggggacggctgccttcgggggggacggggcagggcggggttcggcttctggcgtgtgaccggcggctctagagcctctgctaaccatgttcatgccttcttctttttcctacagctcctgggcaacgtgctggttattgtgctgtctcatcattttggcaaagaattcgccgccaccatggtgtcctattgggatacaggagtgctgctgtgtgctctgctgagctgtctgctgctgacaggctcttcttcaggcaggtaagtttagtctttttgtcttttatttcaggtcccggatccggtggtggtgcaaatcaaagaactgctcctcagtggatgttgcctttacttctagggacacaggcagaccctttgtggagatgtactctgaaatccctgagatcattcacatgacagaaggcagagaactggtgattccctgcagggttaccagcccaaacatcacagtgaccctgaagaagttccccctggacaccctgatccctgatggcaaaagaatcatctgggactctaggaaaggctttatcatctccaatgccacatacaaagagattggcctgctgacctgtgaggctactgtcaatggccacctgtacaaaacaaattacctgacccacagacagaccaacacaatcattgatgtggtgctgagcccatcccatggcattgagctgtctgtgggagaaaagctggtgctgaattgtacagctagaacagaacttaatgtgggcattgatttcaactgggagtaccctagctccaagcaccagcataaaaagctggtgaacagagacctgaagacccagtctggctctgagatgaaaaagttcttgagcaccctgaccattgatggagtgaccagatctgaccagggcctgtacacctgtgctgcctcctctgggctgatgacaaaaaagaacagcacctttgtgagagtgcatgagaaggataaaacccacacctgccctccttgtcctgctcctgagctgctggggggaccatctgtgttcctgttcccccccaagcccaaggataccctgatgatcagcagaaccccagaagtgacctgtgtggtggtggatgtgtcccatgaggacccagaggtgaaattcaactggtatgtggatggagtggaggtgcacaatgccaagaccaaaccaagagaggagcagtataactccacctacagggtggtgtctgtgctgactgtgctgcaccaggattggctgaatggcaaggagtacaagtgcaaggttagcaataaagctctgcctgcccccattgaaaagaccatttccaaagccaaagggcagccaagggagccccaggtgtacaccctgcccccatctagagatgagctgaccaagaaccaggtgagcctcacatgtctggtgaagggcttttacccttctgacattgctgtggagtgggaaagcaatggacagcctgagaataactataagaccacacccccagtgctggattctgatggcagttttttcctgtactctaagctgacagtggacaaatccagatggcagcagggcaatgtgttcagctgctctgtgatgcatgaggccctgcacaatcactatacacagaagagcctgagcctgagcccagggaagtgactcgaggacggggtgaactacgcctgaggatccgatctttttccctctgccaaaaattatggggacatcatgaagccccttgagcatctgacttctggctaataaaggaaatttattttcattgcaatagtgtgttggaattttttgtgtctctcactcggaagcaattcgttgatctgaatttcgaccacccataatacccattaccctggtagataagtagcatggcgggttaatcattaactacaaggaacccctagtgatggagttggccactccctctctgcgcgctcgctcgctcactgaggccgggcgaccaaaggtcgcccgacgcccgggctttgcccgggcggcctcagtgagcgagcgagcgcgcag

SEQ ID NO: 24 - DNA, 3779 bp, synthetic construct
  source 1..3779: mol_type = other DNA
ctgcgcgctcgctcgctcactgaggccgcccgggcaaagcccgggcgtcgggcgacctttggtcgcccggcctcagtgagcgagcgagcgcgcagagagggagtggccaactccatcactaggggttccttgtagttaatgattaacccgccatgctacttatctaccagggtaatggggatcctctagaactatagctagtcgacattgattattgactagttattaatagtaatcaattacggggtcattagttcatagcccatatatggagttccgcgttacataacttacggtaaatggcccgcctggctgaccgcccaacgacccccgcccattgacgtcaataatgacgtatgttcccatagtaacgccaatagggactttccattgacgtcaatgggtggagtatttacggtaaactgcccacttggcagtacatcaagtgtatcatatgccaagtacgccccctattgacgtcaatgacggtaaatggcccgcctggcattatgcccagtacatgaccttatgggactttcctacttggcagtacatctacgtattagtcatcgctattaccatggtcgaggtgagccccacgttctgcttcactctccccatctcccccccctccccacccccaattttgtatttatttattttttaattattttgtgcagcgatgggggcggggggggggggggggcgcgcgccaggcggggcggggcggggcgaggggcggggcggggcgaggcggagaggtgcggcggcagccaatcagagcggcgcgctccgaaagtttccttttatggcgaggcggcggcggcggcggccctataaaaagcgaagcgcgcggcgggcgggagtcgctgcgcgctgccttcgccccgtgccccgctccgccgccgcctcgcgccgcccgccccggctctgactgaccgcgttactcccacaggtgagcgggcgggacggcccttctcctccgggctgtaattagcgcttggtttaatgacggcttgtttcttttctgtggctgcgtgaaagccttgaggggctccgggagggccctttgtgcggggggagcggctcggggggtgcgtgcgtgtgtgtgtgcgtggggagcgccgcgtgcggctccgcgctgcccggcggctgtgagcgctgcgggcgcggcgcggggctttgtgcgctccgcagtgtgcgcgaggggagcgcggccgggggcggtgccccgcggtgcggggggggctgcgaggggaacaaaggctgcgtgcggggtgtgtgcgtgggggggtgagcagggggtgtgggcgcgtcggtcgggctgcaaccccccctgcacccccctccccgagttgctgagcacggcccggcttcgggtgcggggctccgtacggggcgtggcgcggggctcgccgtgccgggcggggggtggcggcaggtgggggtgccgggcggggcggggccgcctcgggccggggagggctcgggggaggggcgcggcggcccccggagcgccggcggctgtcgaggcgcggcgagccgcagccattgccttttatggtaatcgtgcgagagggcgcagggacttcctttgtcccaaatctgtgcggagccgaaatctgggaggcgccgccgcaccccctctagcgggcgcggggcgaagcggtgcggcgccggcaggaaggaaatgggcggggagggccttcgtgcgtcgccgcgccgccgtccccttctccctctccagcctcggggctgtccgcggggggacggctgccttcgggggggacggggcagggcggggttcggcttctggcgtgtgaccggcggctctagagcctctgctaaccatgttcatgccttcttctttttcctacagctcctgggcaacgtgctggttattgtgctgtctcatcattttggcaaagaattcgccgccaccatggtgtcctattgggatacaggagtgctgctgtgtgctctgctgagctgtctgctgctgacaggctcttcttcaggcaggtgagtatctcagggatccagacatggggatatgggaggtgcctctgatcccagggctcactgtgggtctctctgttcacagggacacaggcagaccctttgtggagatgtactctgaaatccctgagatcattcacatgacagaaggcagagaactggtgattccctgcagggttaccagcccaaacatcacagtgaccctgaagaagttccccctggacaccctgatccctgatggcaaaagaatcatctgggactctaggaaaggctttatcatctccaatgccacatacaaagagattggcctgctgacctgtgaggctactgtcaatggccacctgtacaaaacaaattacctgacccacagacagaccaacacaatcattgatgtggtgctgagcccatcccatggcattgagctgtctgtgggagaaaagctggtgctgaattgtacagctagaacagaacttaatgtgggcattgatttcaactgggagtaccctagctccaagcaccagcataaaaagctggtgaacagagacctgaagacccagtctggctctgagatgaaaaagttcttgagcaccctgaccattgatggagtgaccagatctgaccagggcctgtacacctgtgctgcctcctctgggctgatgacaaaaaagaacagcacctttgtgagagtgcatgagaaggataaaacccacacctgccctccttgtcctgctcctgagctgctggggggaccatctgtgttcctgttcccccccaagcccaaggataccctgatgatcagcagaaccccagaagtgacctgtgtggtggtggatgtgtcccatgaggacccagaggtgaaattcaactggtatgtggatggagtggaggtgcacaatgccaagaccaaaccaagagaggagcagtataactccacctacagggtggtgtctgtgctgactgtgctgcaccaggattggctgaatggcaaggagtacaagtgcaaggttagcaataaagctctgcctgcccccattgaaaagaccatttccaaagccaaagggcagccaagggagccccaggtgtacaccctgcccccatctagagatgagctgaccaagaaccaggtgagcctcacatgtctggtgaagggcttttacccttctgacattgctgtggagtgggaaagcaatggacagcctgagaataactataagaccacacccccagtgctggattctgatggcagttttttcctgtactctaagctgacagtggacaaatccagatggcagcagggcaatgtgttcagctgctctgtgatgcatgaggccctgcacaatcactatacacagaagagcctgagcctgagcccagggaagtgactcgaggacggggtgaactacgcctgaggatccgatctttttccctctgccaaaaattatggggacatcatgaagccccttgagcatctgacttctggctaataaaggaaatttattttcattgcaatagtgtgttggaattttttgtgtctctcactcggaagcaattcgttgatctgaatttcgaccacccataatacccattaccctggtagataagtagcatggcgggttaatcattaactacaaggaacccctagtgatggagttggccactccctctctgcgcgctcgctcgctcactgaggccgggcgaccaaaggtcgcccgacgcccgggctttgcccgggcggcctcagtgagcgagcgagcgcgcag

SEQ ID NO: 25 - DNA, 3684 bp, synthetic construct
  source 1..3684: mol_type = other DNA
ctgcgcgctcgctcgctcactgaggccgcccgggcaaagcccgggcgtcgggcgacctttggtcgcccggcctcagtgagcgagcgagcgcgcagagagggagtggccaactccatcactaggggttccttgtagttaatgattaacccgccatgctacttatctaccagggtaatggggatcctctagaactatagctagtcgacattgattattgactagttattaatagtaatcaattacggggtcattagttcatagcccatatatggagttccgcgttacataacttacggtaaatggcccgcctggctgaccgcccaacgacccccgcccattgacgtcaataatgacgtatgttcccatagtaacgccaatagggactttccattgacgtcaatgggtggagtatttacggtaaactgcccacttggcagtacatcaagtgtatcatatgccaagtacgccccctattgacgtcaatgacggtaaatggcccgcctggcattatgcccagtacatgaccttatgggactttcctacttggcagtacatctacgtattagtcatcgctattaccatggtcgaggtgagccccacgttctgcttcactctccccatctcccccccctccccacccccaattttgtatttatttattttttaattattttgtgcagcgatgggggcggggggggggggggggcgcgcgccaggcggggcggggcggggcgaggggcggggcggggcgaggcggagaggtgcggcggcagccaatcagagcggcgcgctccgaaagtttccttttatggcgaggcggcggcggcggcggccctataaaaagcgaagcgcgcggcgggcggggagtcgctgcgacgctgccttcgccccgtgccccgctccgccgccgcctcgcgccgcccgccccggctctgactgaccgcgttactcccacaggtgagcgggcgggacggcccttctcctccgggctgtaattagcgcttggtttaatgacggcttgtttcttttctgtggctgcgtgaaagccttgaggggctccgggagggccctttgtgcggggggagcggctcggggggtgcgtgcgtgtgtgtgtgcgtggggagcgccgcgtgcggctccgcgctgcccggcggctgtgagcgctgcgggcgcggcgcggggctttgtgcgctccgcagtgtgcgcgaggggagcgcggccgggggcggtgccccgcggtgcggggggggctgcgaggggaacaaaggctgcgtgcggggtgtgtgcgtgggggggtgagcagggggtgtgggcgcgtcggtcgggctgcaaccccccctgcacccccctccccgagttgctgagcacggcccggcttcgggtgcggggctccgtacggggcgtggcgcggggctcgccgtgccgggcggggggtggcggcaggtgggggtgccgggcggggcggggccgcctcgggccggggagggctcgggggaggggcgcggcggcccccggagcgccggcggctgtcgaggcgcggcgagccgcagccattgccttttatggtaatcgtgcgagagggcgcagggacttcctttgtcccaaatctgtgcggagccgaaatctgggaggcgccgccgcaccccctctagcgggcgcggggcgaagcggtgcggcgccggcaggaaggaaatgggcggggagggccttcgtgcgtcgccgcgccgccgtccccttctccctctccagcctcggggctgtccgcggggggacggctgccttcgggggggacggggcagggcggggttcggcttctggcgtgtgaccggcggctctagagcctctgctaaccatgttcatgccttcttctttttcctacagctcctgggcaacgtgctggttattgtgctgtctcatcattttggcaaagaattcgccgccaccatgatgtacagaatgcagctgctgctgctgatcgccctgagcctggccctggtgaccaacagcagcgacaccggtagacctttcgtagagatgtacagtgaaatccccgaaattatacacatgactgaaggaagggagctcgtcattccctgccgggttacgtcacctaacatcactgttactttaaaaaagtttccacttgacactttgatccctgatggaaaacgcataatctgggacagtagaaagggcttcatcatatcaaatgcaacgtacaaagaaatagggcttctgacctgtgaagcaacagtcaatgggcatttgtataagacaaactatctcacacatcgacaaaccaatacaatcatagatgtggttctgagtccgtctcatggaattgaactatctgttggagaaaagcttgtcttaaattgtacagcaagaactgaactaaatgtggggattgacttcaactgggaatacccttcttcgaagcatcagcataagaaacttgtaaaccgagacctaaaaacccagtctgggagtgagatgaagaaatttttgagcaccttaactatagatggtgtaacccggagtgaccaaggattgtacacctgtgcagcatccagtgggctgatgaccaagaagaacagcacatttgtcagggtccatgaaaaagacaaaactcacacatgcccaccgtgcccagcacctgaactcctggggggaccgtcagtcttcctcttccccccaaaacccaaggacaccctcatgatctcccggacccctgaggtcacatgcgtggtggtggacgtgagccacgaagaccctgaggtcaagttcaactggtacgtggacggcgtggaggtgcataatgccaagacaaagccgcgggaggagcagtacaacagcacgtaccgtgtggtcagcgtcctcaccgtcctgcaccaggactggctgaatggcaaggagtacaagtgcaaggtctccaacaaagccctcccagcccccatcgagaaaaccatctccaaagccaaagggcagccccgagaaccacaggtgtacaccctgcccccatcccgggatgagctgaccaagaaccaggtcagcctgacctgcctggtcaaaggcttctatcccagcgacatcgccgtggagtgggagagcaatgggcagccggagaacaactacaagaccacgcctcccgtgctggactccgacggctccttcttcctctatagcaagctcaccgtggacaagagcaggtggcagcaggggaacgtcttctcatgctccgtgatgcatgaggctctgcacaaccactacacgcagaagagcctctccctgtctccgggtaaataactcgaggacggggtgaactacgcctgaggatccgatctttttccctctgccaaaaattatggggacatcatgaagccccttgagcatctgacttctggctaataaaggaaatttattttcattgcaatagtgtgttggaattttttgtgtctctcactcggaagcaattcgttgatctgaatttcgaccacccataatacccattaccctggtagataagtagcatggcgggttaatcattaactacaaggaacccctagtgatggagttggccactccctctctgcgcgctcgctcgctcactgaggccgggcgaccaaaggtcgcccgacgcccgggctttgcccgggcggcctcagtgagcgagcgagcgcgcag

SEQ ID NO: 26 - DNA, 6434 bp, synthetic construct
  source 1..6434: mol_type = other DNA
ctcgaggacggggtgaactacgcctgaggatccgatctttttccctctgccaaaaattatggggacatcatgaagccccttgagcatctgacttctggctaataaaggaaatttattttcattgcaatagtgtgttggaattttttgtgtctctcactcggaagcaattcgttgatctgaatttcgaccacccataatacccattaccctggtagataagtagcatggcgggttaatcattaactacaaggaacccctagtgatggagttggccactccctctctgcgcgctcgctcgctcactgaggccgggcgaccaaaggtcgcccgacgcccgggctttgcccgggcggcctcagtgagcgagcgagcgcgcagccttaattaacctaattcactggccgtcgttttacaacgtcgtgactgggaaaaccctggcgttacccaacttaatcgccttgcagcacatccccctttcgccagctggcgtaatagcgaagaggcccgcaccgatcgcccttcccaacagttgcgcagcctgaatggcgaatgggacgcgccctgtagcggcgcattaagcgcggcgggtgtggtggttacgcgcagcgtgaccgctacacttgccagcgccctagcgcccgctcctttcgctttcttcccttcctttctcgccacgttcgccggctttccccgtcaagctctaaatcgggggctccctttagggttccgatttagtgctttacggcacctcgaccccaaaaaacttgattagggtgatggttcacgtagtgggccatcgccctgatagacggtttttcgccctttgacgttggagtccacgttctttaatagtggactcttgttccaaactggaacaacactcaaccctatctcggtctattcttttgatttataagggattttgccgatttcggcctattggttaaaaaatgagctgatttaacaaaaatttaacgcgaattttaacaaaatattaacgcttacaatttaggtggcacttttcggggaaatgtgcgcggaacccctatttgtttatttttctaaatacattcaaatatgtatccgctcatgagacaataaccctgataaatgcttcaataatattgaaaaaggaagagtatgattgaacaagatggattgcacgcaggttctccggccgcttgggtggagaggctattcggctatgactgggcacaacagacaatcggctgctctgatgccgccgtgttccggctgtcagcgcaggggcgcccggttctttttgtcaagaccgacctgtccggtgccctgaatgaactgcaagacgaggcagcgcggctatcgtggctggccacgacgggcgttccttgcgcagctgtgctcgacgttgtcactgaagcgggaagggactggctgctattgggcgaagtgccggggcaggatctcctgtcatctcaccttgctcctgccgagaaagtatccatcatggctgatgcaatgcggcggctgcatacgcttgatccggctacctgcccattcgaccaccaagcgaaacatcgcatcgagcgagcacgtactcggatggaagccggtcttgtcgatcaggatgatctggacgaagagcatcaggggctcgcgccagccgaactgttcgccaggctcaaggcgagcatgcccgacggcgaggatctcgtcgtgacccatggcgatgcctgcttgccgaatatcatggtggaaaatggccgcttttctggattcatcgactgtggccggctgggtgtggcggaccgctatcaggacatagcgttggctacccgtgatattgctgaagagcttggcggcgaatgggctgaccgcttcctcgtgctttacggtatcgccgctcccgattcgcagcgcatcgccttctatcgccttcttgacgagttcttctgactgtcagaccaagtttactcatatatactttagattgatttaaaacttcatttttaatttaaaaggatctaggtgaagatcctttttgataatctcatgaccaaaatcccttaacgtgagttttcgttccactgagcgtcagaccccgtagaaaagatcaaaggatcttcttgagatcctttttttctgcgcgtaatctgctgcttgcaaacaaaaaaaccaccgctaccagcggtggtttgtttgccggatcaagagctaccaactctttttccgaaggtaactggcttcagcagagcgcagataccaaatactgttcttctagtgtagccgtagttaggccaccacttcaagaactctgtagcaccgcctacatacctcgctctgctaatcctgttaccagtggctgctgccagtggcgataagtcgtgtcttaccgggttggactcaagacgatagttaccggataaggcgcagcggtcgggctgaacggggggttcgtgcacacagcccagcttggagcgaacgacctacaccgaactgagatacctacagcgtgagctatgagaaagcgccacgcttcccgaagggagaaaggcggacaggtatccggtaagcggcagggtcggaacaggagagcgcacgagggagcttccagggggaaacgcctggtatctttatagtcctgtcgggtttcgccacctctgacttgagcgtcgatttttgtgatgctcgtcaggggggcggagcctatggaaaaacgccagcaacgcggcctttttacggttcctggccttttgctggccttttgctcacatgttctttcctgcgttatcccctgattctgtggataaccgtattaccgcctttgagtgagctgataccgctcgccgcagccgaacgaccgagcgcagcgagtcagtgagcgaggaagcggaagagcgcccaatacgcaaaccgcctctccccgcgcgttggccgattcattaatgcagctggcacgacaggtttcccgactggaaagcgggcagtgagcgcaacgcaattaatgtgagttagctcactcattaggcaccccaggctttacactttatgcttccggctcgtatgttgtgtggaattgtgagcggataacaatttcacacaggaaacagctatgaccatgattacgccagatttaattaaggccttaattaggctgcgcgctcgctcgctcactgaggccgcccgggcaaagcccgggcgtcgggcgacctttggtcgcccggcctcagtgagcgagcgagcgcgcagagagggagtggccaactccatcactaggggttccttgtagttaatgattaacccgccatgctacttatctaccagggtaatggggatcctctagaactatagctagtcgacattgattattgactagttattaatagtaatcaattacggggtcattagttcatagcccatatatggagttccgcgttacataacttacggtaaatggcccgcctggctgaccgcccaacgacccccgcccattgacgtcaataatgacgtatgttcccatagtaacgccaatagggactttccattgacgtcaatgggtggagtatttacggtaaactgcccacttggcagtacatcaagtgtatcatatgccaagtacgccccctattgacgtcaatgacggtaaatggcccgcctggcattatgcccagtacatgaccttatgggactttcctacttggcagtacatctacgtattagtcatcgctattaccatggtcgaggtgagccccacgttctgcttcactctccccatctcccccccctccccacccccaattttgtatttatttattttttaattattttgtgcagcgatgggggcggggggggggggggggcgcgcgccaggcggggcggggcggggcgaggggcggggcggggcaaggcggagaggtgcggcggcagccaatcagagcggcgcgctccgaaagtttccttttatggcgaggcggcggcggcggcggccctataaaaagcgaagcgcgcggcgggcgggagtcgctgcgcgctgccttcgccccgtgccccgctccgccgccgcctcgcgccgcccgccccggctctgactgaccgcgttactcccacaggtgagcgggcgggacggcccttctcctccgggctgtaattagcgcttggtttaatgacggcttgtttcttttctgtggctgcgtgaaagccttgaggggctccgggagggccctttgtgcggggggagcggctcggggggtgcgtgcgtgtgtgtgtgcgtggggagcgccgcgtgcggctccgcgctgcccggcggctgtgagcgctgcgggcgcggcgcggggctttgtgcgctccgcagtgtgcgcgaggggagcgcggccgggggcggtgccccgcggtgcggggggggctgcgaggggaacaaaggctgcgtgcggggtgtgtgcgtgggggggtgagcagggggtgtgggcgcgtcggtcgggctgcaaccccccctgcacccccctccccgagttgctgagcacggcccggcttcgggtgcggggctccgtacggggcgtggcgcggggctcgccgtgccgggcggggggtggcggcaggtgggggtgccgggcggggcggggccgcctcgggccggggagggctcgggggaggggcgcggcggcccccggagcgccggcggctgtcgaggcgcggcgagccgcagccattgccttttatggtaatcgtgcgagagggcgcagggacttcctttgtcccaaatctgtgcggagccgaaatctgggaggcgccgccgcaccccctctagcgggcgcggggcgaagcggtgcggcgccggcaggaaggaaatgggcggggagggccttcgtgcgtcgccgcgccgccgtccccttctccctctccagcctcggggctgtccgcggggggacggctgccttcgggggggacggggcagggcggggttcggcttctggcgtgtgaccggcggctctagagcctctgctaaccatgttcatgccttcttctttttcctacagctcctgggcaacgtgctggttattgtgctgtctcatcattttggcaaagaattcgccgccaccatgtacagaatgcagctgctgctgctgatcgccctgagcctggccctggtgaccaacagcagcgacaccggtagacctttcgtagagatgtacagtgaaatccccgaaattatacacatgactgaaggaagggagctcgtcattccctgccgggttacgtcacctaacatcactgttactttaaaaaagtttccacttgacactttgatccctgatggaaaacgcataatctgggacagtagaaagggcttcatcatatcaaatgcaacgtacaaagaaatagggcttctgacctgtgaagcaacagtcaatgggcatttgtataagacaaactatctcacacatcgacaaaccaatacaatcatagatgtggttctgagtccgtctcatggaattgaactatctgttggagaaaagcttgtcttaaattgtacagcaagaactgaactaaatgtggggattgacttcaactgggaatacccttcttcgaagcatcagcataagaaacttgtaaaccgagacctaaaaacccagtctgggagtgagatgaagaaatttttgagcaccttaactatagatggtgtaacccggagtgaccaaggattgtacacctgtgcagcatccagtgggctgatgaccaagaagaacagcacatttgtcagggtccatgaaaaagacaaaactcacacatgcccaccgtgcccagcacctgaactcctggggggaccgtcagtcttcctcttccccccaaaacccaaggacaccctcatgatctcccggacccctgaggtcacatgcgtggtggtggacgtgagccacgaagaccctgaggtcaagttcaactggtacgtggacggcgtggaggtgcataatgccaagacaaagccgcgggaggagcagtacaacagcacgtaccgtgtggtcagcgtcctcaccgtcctgcaccaggactggctgaatggcaaggagtacaagtgcaaggtctccaacaaagccctcccagcccccatcgagaaaaccatctccaaagccaaagggcagccccgagaaccacaggtgtacaccctgcccccatcccgggatgagctgaccaagaaccaggtcagcctgacctgcctggtcaaaggcttctatcccagcgacatcgccgtggagtgggagagcaatgggcagccggagaacaactacaagaccacgcctcccgtgctggactccgacggctccttcttcctctatagcaagctcaccgtggacaagagcaggtggcagcaggggaacgtcttctcatgctccgtgatgcatgaggctctgcacaaccactacacgcagaagagcctctccctgtctccgggtaaataa

SEQ ID NO: 27 - DNA, 3699 bp, synthetic construct
  source 1..3699: mol_type = other DNA
ctgcgcgctcgctcgctcactgaggccgcccgggcaaagcccgggcgtcgggcgacctttggtcgcccggcctcagtgagcgagcgagcgcgcagagagggagtggccaactccatcactaggggttccttgtagttaatgattaacccgccatgctacttatctaccagggtaatggggatcctctagaactatagctagtcgacattgattattgactagttattaatagtaatcaattacggggtcattagttcatagcccatatatggagttccgcgttacataacttacggtaaatggcccgcctggctgaccgcccaacgacccccgcccattgacgtcaataatgacgtatgttcccatagtaacgccaatagggactttccattgacgtcaatgggtggagtatttacggtaaactgcccacttggcagtacatcaagtgtatcatatgccaagtacgccccctattgacgtcaatgacggtaaatggcccgcctggcattatgcccagtacatgaccttatgggactttcctacttggcagtacatctacgtattagtcatcgctattaccatggtcgaggtgagccccacgttctgcttcactctccccatctcccccccctccccacccccaattttgtatttatttattttttaattattttgtgcagcgatgggggcggggggggggggggggcgcgcgccaggcggggcggggcggggcgaggggcggggcggggcgaggcggagaggtgcggcggcagccaatcagagcggcgcgctccgaaagtttccttttatggcgaggcggcggcggcggcggccctataaaaagcgaagcgcgcggcgggcggggagtcgctgcgacgctgccttcgccccgtgccccgctccgccgccgcctcgcgccgcccgccccggctctgactgaccgcgttactcccacaggtgagcgggcgggacggcccttctcctccgggctgtaattagcgcttggtttaatgacggcttgtttcttttctgtggctgcgtgaaagccttgaggggctccgggagggccctttgtgcggggggagcggctcggggggtgcgtgcgtgtgtgtgtgcgtggggagcgccgcgtgcggctccgcgctgcccggcggctgtgagcgctgcgggcgcggcgcggggctttgtgcgctccgcagtgtgcgcgaggggagcgcggccgggggcggtgccccgcggtgcggggggggctgcgaggggaacaaaggctgcgtgcggggtgtgtgcgtgggggggtgagcagggggtgtgggcgcgtcggtcgggctgcaaccccccctgcacccccctccccgagttgctgagcacggcccggcttcgggtgcggggctccgtacggggcgtggcgcggggctcgccgtgccgggcggggggtggcggcaggtgggggtgccgggcggggcggggccgcctcgggccggggagggctcgggggaggggcgcggcggcccccggagcgccggcggctgtcgaggcgcggcgagccgcagccattgccttttatggtaatcgtgcgagagggcgcagggacttcctttgtcccaaatctgtgcggagccgaaatctgggaggcgccgccgcaccccctctagcgggcgcggggcgaagcggtgcggcgccggcaggaaggaaatgggcggggagggccttcgtgcgtcgccgcgccgccgtccccttctccctctccagcctcggggctgtccgcggggggacggctgccttcgggggggacggggcagggcggggttcggcttctggcgtgtgaccggcggctctagagcctctgctaaccatgttcatgccttcttctttttcctacagctcctgggcaacgtgctggttattgtgctgtctcatcattttggcaaagaattcgccgccaccatggtgtcctattgggataccggagtgctgctgtgcgctctgctgagctgtctgctgctgacaggctcttcttcaggcagcgacaccggccggcccttcgtggagatgtacagcgaaatccctgagatcattcacatgacagaaggccgcgaactggtgattccctgcagggttaccagcccaaacatcaccgtgaccctgaagaagttccccctggacaccctgatccctgacggcaaacggatcatctgggactctaggaaaggctttatcatctccaatgccacatacaaagagattggcctgctgacctgcgaggctacggtcaacggccacctgtacaaaacaaattacctgacccacagacagaccaacacaatcatcgacgtggtgctgagcccatcccatggcattgagctgtccgtgggagaaaagctggtgctgaattgtacggctagaacagaacttaacgtgggcatcgatttcaactgggagtaccctagctccaagcaccagcataaaaagctggtgaaccgggacctgaagacccagtccggcagtgagatgaaaaagttcttgagcaccctgaccatcgatggagtgacccgaagcgaccagggcctgtacacctgtgccgcctcctctgggctgatgacaaaaaagaacagcacctttgtcagagtgcacgagaaggataaaacccacacctgccctccttgtcccgctcctgagctgctggggggaccatctgtgttcctgttcccccccaagcccaaggataccctgatgatcagccgaaccccagaagtgacctgcgtggtggtggacgtgtcccacgaggacccagaggtgaaattcaactggtatgtggacggcgtggaggtgcacaatgccaagaccaaaccaagagaggagcagtataactccacctacagggtggtgagcgtgctgactgtgctgcaccaggattggctgaacggcaaggagtacaagtgcaaggttagcaataaagctctgcccgcccccatcgaaaagaccatttccaaagccaaagggcagccaagggagccccaggtgtacaccctgcccccatctcgggacgagctgaccaagaaccaggtgagtctcacatgtctcgtgaagggcttttaccctagcgacatcgccgtcgagtgggaaagcaacggacagcctgagaataactataagaccacaccccccgtgctggattccgacggcagttttttcctgtactctaagctgacagtggacaaatcccgctggcagcagggcaacgtgttcagctgctccgtgatgcacgaggccctgcacaatcactatacacagaagagcctgagcctgagccccgggaagtgactcgaggacggggtgaactacgcctgaggatccgatctttttccctctgccaaaaattatggggacatcatgaagccccttgagcatctgacttctggctaataaaggaaatttattttcattgcaatagtgtgttggaattttttgtgtctctcactcggaagcaattcgttgatctgaatttcgaccacccataatacccattaccctggtagataagtagcatggcgggttaatcattaactacaaggaacccctagtgatggagttggccactccctctctgcgcgctcgctcgctcactgaggccgggcgaccaaaggtcgcccgacgcccgggctttgcccgggcggcctcagtgagcgagcgagcgcgcag

SEQ ID NO: 28 - DNA, 6452 bp, synthetic construct
  source 1..6452: mol_type = other DNA
ctcgaggacggggtgaactacgcctgaggatccgatctttttccctctgccaaaaattatggggacatcatgaagccccttgagcatctgacttctggctaataaaggaaatttattttcattgcaatagtgtgttggaattttttgtgtctctcactcggaagcaattcgttgatctgaatttcgaccacccataatacccattaccctggtagataagtagcatggcgggttaatcattaactacaaggaacccctagtgatggagttggccactccctctctgcgcgctcgctcgctcactgaggccgggcgaccaaaggtcgcccgacgcccgggctttgcccgggcggcctcagtgagcgagcgagcgcgcagccttaattaacctaattcactggccgtcgttttacaacgtcgtgactgggaaaaccctggcgttacccaacttaatcgccttgcagcacatccccctttcgccagctggcgtaatagcgaagaggcccgcaccgatcgcccttcccaacagttgcgcagcctgaatggcgaatgggacgcgccctgtagcggcgcattaagcgcggcgggtgtggtggttacgcgcagcgtgaccgctacacttgccagcgccctagcgcccgctcctttcgctttcttcccttcctttctcgccacgttcgccggctttccccgtcaagctctaaatcgggggctccctttagggttccgatttagtgctttacggcacctcgaccccaaaaaacttgattagggtgatggttcacgtagtgggccatcgccctgatagacggtttttcgccctttgacgttggagtccacgttctttaatagtggactcttgttccaaactggaacaacactcaaccctatctcggtctattcttttgatttataagggattttgccgatttcggcctattggttaaaaaatgagctgatttaacaaaaatttaacgcgaattttaacaaaatattaacgcttacaatttaggtggcacttttcggggaaatgtgcgcggaacccctatttgtttatttttctaaatacattcaaatatgtatccgctcatgagacaataaccctgataaatgcttcaataatattgaaaaaggaagagtatgattgaacaagatggattgcacgcaggttctccggccgcttgggtggagaggctattcggctatgactgggcacaacagacaatcggctgctctgatgccgccgtgttccggctgtcagcgcaggggcgcccggttctttttgtcaagaccgacctgtccggtgccctgaatgaactgcaagacgaggcagcgcggctatcgtggctggccacgacgggcgttccttgcgcagctgtgctcgacgttgtcactgaagcgggaagggactggctgctattgggcgaagtgccggggcaggatctcctgtcatctcaccttgctcctgccgagaaagtatccatcatggctgatgcaatgcggcggctgcatacgcttgatccggctacctgcccattcgaccaccaagcgaaacatcgcatcgagcgagcacgtactcggatggaagccggtcttgtcgatcaggatgatctggacgaagagcatcaggggctcgcgccagccgaactgttcgccaggctcaaggcgagcatgcccgacggcgaggatctcgtcgtgacccatggcgatgcctgcttgccgaatatcatggtggaaaatggccgcttttctggattcatcgactgtggccggctgggtgtggcggaccgctatcaggacatagcgttggctacccgtgatattgctgaagagcttggcggcgaatgggctgaccgcttcctcgtgctttacggtatcgccgctcccgattcgcagcgcatcgccttctatcgccttcttgacgagttcttctgactgtcagaccaagtttactcatatatactttagattgatttaaaacttcatttttaatttaaaaggatctaggtgaagatcctttttgataatctcatgaccaaaatcccttaacgtgagttttcgttccactgagcgtcagaccccgtagaaaagatcaaaggatcttcttgagatcctttttttctgcgcgtaatctgctgcttgcaaacaaaaaaaccaccgctaccagcggtggtttgtttgccggatcaagagctaccaactctttttccgaaggtaactggcttcagcagagcgcagataccaaatactgttcttctagtgtagccgtagttaggccaccacttcaagaactctgtagcaccgcctacatacctcgctctgctaatcctgttaccagtggctgctgccagtggcgataagtcgtgtcttaccgggttggactcaagacgatagttaccggataaggcgcagcggtcgggctgaacggggggttcgtgcacacagcccagcttggagcgaacgacctacaccgaactgagatacctacagcgtgagctatgagaaagcgccacgcttcccgaagggagaaaggcggacaggtatccggtaagcggcagggtcggaacaggagagcgcacgagggagcttccagggggaaacgcctggtatctttatagtcctgtcgggtttcgccacctctgacttgagcgtcgatttttgtgatgctcgtcaggggggcggagcctatggaaaaacgccagcaacgcggcctttttacggttcctggccttttgctggccttttgctcacatgttctttcctgcgttatcccctgattctgtggataaccgtattaccgcctttgagtgagctgataccgctcgccgcagccgaacgaccgagcgcagcgagtcagtgagcgaggaagcggaagagcgcccaatacgcaaaccgcctctccccgcgcgttggccgattcattaatgcagctggcacgacaggtttcccgactggaaagcgggcagtgagcgcaacgcaattaatgtgagttagctcactcattaggcaccccaggctttacactttatgcttccggctcgtatgttgtgtggaattgtgagcggataacaatttcacacaggaaacagctatgaccatgattacgccagatttaattaaggccttaattaggctgcgcgctcgctcgctcactgaggccgcccgggcaaagcccgggcgtcgggcgacctttggtcgcccggcctcagtgagcgagcgagcgcgcagagagggagtggccaactccatcactaggggttccttgtagttaatgattaacccgccatgctacttatctaccagggtaatggggatcctctagaactatagctagtcgacattgattattgactagttattaatagtaatcaattacggggtcattagttcatagcccatatatggagttccgcgttacataacttacggtaaatggcccgcctggctgaccgcccaacgacccccgcccattgacgtcaataatgacgtatgttcccatagtaacgccaatagggactttccattgacgtcaatgggtggagtatttacggtaaactgcccacttggcagtacatcaagtgtatcatatgccaagtacgccccctattgacgtcaatgacggtaaatggcccgcctggcattatgcccagtacatgaccttatgggactttcctacttggcagtacatctacgtattagtcatcgctattaccatggtcgaggtgagccccacgttctgcttcactctccccatctcccccccctccccacccccaattttgtatttatttattttttaattattttgtgcagcgatgggggcggggggggggggggggcgcgcgccaggcggggcggggcggggcgaggggcggggcggggcaaggcggagaggtgcggcggcagccaatcagagcggcgcgctccgaaagtttccttttatggcgaggcggcggcggcggcggccctataaaaagcgaagcgcgcggcgggcgggagtcgctgcgcgctgccttcgccccgtgccccgctccgccgccgcctcgcgccgcccgccccggctctgactgaccgcgttactcccacaggtgagcgggcgggacggcccttctcctccgggctgtaattagcgcttggtttaatgacggcttgtttcttttctgtggctgcgtgaaagccttgaggggctccgggagggccctttgtgcggggggagcggctcggggggtgcgtgcgtgtgtgtgtgcgtggggagcgccgcgtgcggctccgcgctgcccggcggctgtgagcgctgcgggcgcggcgcggggctttgtgcgctccgcagtgtgcgcgaggggagcgcggccgggggcggtgccccgcggtgcggggggggctgcgaggggaacaaaggctgcgtgcggggtgtgtgcgtgggggggtgagcagggggtgtgggcgcgtcggtcgggctgcaaccccccctgcacccccctccccgagttgctgagcacggcccggcttcgggtgcggggctccgtacggggcgtggcgcggggctcgccgtgccgggcggggggtggcggcaggtgggggtgccgggcggggcggggccgcctcgggccggggagggctcgggggaggggcgcggcggcccccggagcgccggcggctgtcgaggcgcggcgagccgcagccattgccttttatggtaatcgtgcgagagggcgcagggacttcctttgtcccaaatctgtgcggagccgaaatctgggaggcgccgccgcaccccctctagcgggcgcggggcgaagcggtgcggcgccggcaggaaggaaatgggcggggagggccttcgtgcgtcgccgcgccgccgtccccttctccctctccagcctcggggctgtccgcggggggacggctgccttcgggggggacggggcagggcggggttcggcttctggcgtgtgaccggcggctctagagcctctgctaaccatgttcatgccttcttctttttcctacagctcctgggcaacgtgctggttattgtgctgtctcatcattttggcaaagaattcgccgccaccatggtgtcctattgggataccggagtgctgctgtgcgctctgctgagctgtctgctgctgacaggctcttcttcaggcagcgacaccggccggcccttcgtggagatgtacagcgaaatccctgagatcattcacatgacagaaggccgcgaactggtgattccctgcagggttaccagcccaaacatcaccgtgaccctgaagaagttccccctggacaccctgatccctgacggcaaacggatcatctgggactctaggaaaggctttatcatctccaatgccacatacaaagagattggcctgctgacctgcgaggctacggtcaacggccacctgtacaaaacaaattacctgacccacagacagaccaacacaatcatcgacgtggtgctgagcccatcccatggcattgagctgtccgtgggagaaaagctggtgctgaattgtacggctagaacagaacttaacgtgggcatcgatttcaactgggagtaccctagctccaagcaccagcataaaaagctggtgaaccgggacctgaagacccagtccggcagtgagatgaaaaagttcttgagcaccctgaccatcgatggagtgacccgaagcgaccagggcctgtacacctgtgccgcctcctctgggctgatgacaaaaaagaacagcacctttgtcagagtgcacgagaaggataaaacccacacctgccctccttgtcccgctcctgagctgctggggggaccatctgtgttcctgttcccccccaagcccaaggataccctgatgatcagccgaaccccagaagtgacctgcgtggtggtggacgtgtcccacgaggacccagaggtgaaattcaactggtatgtggacggcgtggaggtgcacaatgccaagaccaaaccaagagaggagcagtataactccacctacagggtggtgagcgtgctgactgtgctgcaccaggattggctgaacggcaaggagtacaagtgcaaggttagcaataaagctctgcccgcccccatcgaaaagaccatttccaaagccaaagggcagccaagggagccccaggtgtacaccctgcccccatctcgggacgagctgaccaagaaccaggtgagtctcacatgtctcgtgaagggcttttaccctagcgacatcgccgtcgagtgggaaagcaacggacagcctgagaataactataagaccacaccccccgtgctggattccgacggcagttttttcctgtactctaagctgacagtggacaaatcccgctggcagcagggcaacgtgttcagctgctccgtgatgcacgaggccctgcacaatcactatacacagaagagcctgagcctgagccccgggaagtga

SEQ ID NO: 29 - DNA, 3699 bp, synthetic construct
  source 1..3699: mol_type = other DNA
ctgcgcgctcgctcgctcactgaggccgcccgggcaaagcccgggcgtcgggcgacctttggtcgcccggcctcagtgagcgagcgagcgcgcagagagggagtggccaactccatcactaggggttccttgtagttaatgattaacccgccatgctacttatctaccagggtaatggggatcctctagaactatagctagtcgacattgattattgactagttattaatagtaatcaattacggggtcattagttcatagcccatatatggagttccgcgttacataacttacggtaaatggcccgcctggctgaccgcccaacgacccccgcccattgacgtcaataatgacgtatgttcccatagtaacgccaatagggactttccattgacgtcaatgggtggagtatttacggtaaactgcccacttggcagtacatcaagtgtatcatatgccaagtacgccccctattgacgtcaatgacggtaaatggcccgcctggcattatgcccagtacatgaccttatgggactttcctacttggcagtacatctacgtattagtcatcgctattaccatggtcgaggtgagccccacgttctgcttcactctccccatctcccccccctccccacccccaattttgtatttatttattttttaattattttgtgcagcgatgggggcggggggggggggggggcgcgcgccaggcggggcggggcggggcgaggggcggggcggggcgaggcggagaggtgcggcggcagccaatcagagcggcgcgctccgaaagtttccttttatggcgaggcggcggcggcggcggccctataaaaagcgaagcgcgcggcgggcggggagtcgctgcgacgctgccttcgccccgtgccccgctccgccgccgcctcgcgccgcccgccccggctctgactgaccgcgttactcccacaggtgagcgggcgggacggcccttctcctccgggctgtaattagcgcttggtttaatgacggcttgtttcttttctgtggctgcgtgaaagccttgaggggctccgggagggccctttgtgcggggggagcggctcggggggtgcgtgcgtgtgtgtgtgcgtggggagcgccgcgtgcggctccgcgctgcccggcggctgtgagcgctgcgggcgcggcgcggggctttgtgcgctccgcagtgtgcgcgaggggagcgcggccgggggcggtgccccgcggtgcggggggggctgcgaggggaacaaaggctgcgtgcggggtgtgtgcgtgggggggtgagcagggggtgtgggcgcgtcggtcgggctgcaaccccccctgcacccccctccccgagttgctgagcacggcccggcttcgggtgcggggctccgtacggggcgtggcgcggggctcgccgtgccgggcggggggtggcggcaggtgggggtgccgggcggggcggggccgcctcgggccggggagggctcgggggaggggcgcggcggcccccggagcgccggcggctgtcgaggcgcggcgagccgcagccattgccttttatggtaatcgtgcgagagggcgcagggacttcctttgtcccaaatctgtgcggagccgaaatctgggaggcgccgccgcaccccctctagcgggcgcggggcgaagcggtgcggcgccggcaggaaggaaatgggcggggagggccttcgtgcgtcgccgcgccgccgtccccttctccctctccagcctcggggctgtccgcggggggacggctgccttcgggggggacggggcagggcggggttcggcttctggcgtgtgaccggcggctctagagcctctgctaaccatgttcatgccttcttctttttcctacagctcctgggcaacgtgctggttattgtgctgtctcatcattttggcaaagaattcgccgccaccatggtgtcctattgggatacaggagtgctgctgtgtgctctgctgagctgtctgctgctgacaggctcttcttcaggctctgacacaggcagaccctttgtggagatgtactctgaaatccctgagatcattcacatgacagaaggcagagaactggtgattccctgcagggttaccagcccaaacatcacagtgaccctgaagaagttccccctggacaccctgatccctgatggcaaaagaatcatctgggactctaggaaaggctttatcatctccaatgccacatacaaagagattggcctgctgacctgtgaggctactgtcaatggccacctgtacaaaacaaattacctgacccacagacagaccaacacaatcattgatgtggtgctgagcccatcccatggcattgagctgtctgtgggagaaaagctggtgctgaattgtacagctagaacagaacttaatgtgggcattgatttcaactgggagtaccctagctccaagcaccagcataaaaagctggtgaacagagacctgaagacccagtctggctctgagatgaaaaagttcttgagcaccctgaccattgatggagtgaccagatctgaccagggcctgtacacctgtgctgcctcctctgggctgatgacaaaaaagaacagcacctttgtgagagtgcatgagaaggataaaacccacacctgccctccttgtcctgctcctgagctgctggggggaccatctgtgttcctgttcccccccaagcccaaggataccctgatgatcagcagaaccccagaagtgacctgtgtggtggtggatgtgtcccatgaggacccagaggtgaaattcaactggtatgtggatggagtggaggtgcacaatgccaagaccaaaccaagagaggagcagtataactccacctacagggtggtgtctgtgctgactgtgctgcaccaggattggctgaatggcaaggagtacaagtgcaaggttagcaataaagctctgcctgcccccattgaaaagaccatttccaaagccaaagggcagccaagggagccccaggtgtacaccctgcccccatctagagatgagctgaccaagaaccaggtgagcctcacatgtctggtgaagggcttttacccttctgacattgctgtggagtgggaaagcaatggacagcctgagaataactataagaccacacccccagtgctggattctgatggcagttttttcctgtactctaagctgacagtggacaaatccagatggcagcagggcaatgtgttcagctgctctgtgatgcatgaggccctgcacaatcactatacacagaagagcctgagcctgagcccagggaagtgactcgaggacggggtgaactacgcctgaggatccgatctttttccctctgccaaaaattatggggacatcatgaagccccttgagcatctgacttctggctaataaaggaaatttattttcattgcaatagtgtgttggaattttttgtgtctctcactcggaagcaattcgttgatctgaatttcgaccacccataatacccattaccctggtagataagtagcatggcgggttaatcattaactacaaggaacccctagtgatggagttggccactccctctctgcgcgctcgctcgctcactgaggccgggcgaccaaaggtcgcccgacgcccgggctttgcccgggcggcctcagtgagcgagcgagcgcgcag

SEQ ID NO: 30 - DNA, 6452 bp, synthetic construct
  source 1..6452: mol_type = other DNA
ctcgaggacggggtgaactacgcctgaggatccgatctttttccctctgccaaaaattatggggacatcatgaagccccttgagcatctgacttctggctaataaaggaaatttattttcattgcaatagtgtgttggaattttttgtgtctctcactcggaagcaattcgttgatctgaatttcgaccacccataatacccattaccctggtagataagtagcatggcgggttaatcattaactacaaggaacccctagtgatggagttggccactccctctctgcgcgctcgctcgctcactgaggccgggcgaccaaaggtcgcccgacgcccgggctttgcccgggcggcctcagtgagcgagcgagcgcgcagccttaattaacctaattcactggccgtcgttttacaacgtcgtgactgggaaaaccctggcgttacccaacttaatcgccttgcagcacatccccctttcgccagctggcgtaatagcgaagaggcccgcaccgatcgcccttcccaacagttgcgcagcctgaatggcgaatgggacgcgccctgtagcggcgcattaagcgcggcgggtgtggtggttacgcgcagcgtgaccgctacacttgccagcgccctagcgcccgctcctttcgctttcttcccttcctttctcgccacgttcgccggctttccccgtcaagctctaaatcgggggctccctttagggttccgatttagtgctttacggcacctcgaccccaaaaaacttgattagggtgatggttcacgtagtgggccatcgccctgatagacggtttttcgccctttgacgttggagtccacgttctttaatagtggactcttgttccaaactggaacaacactcaaccctatctcggtctattcttttgatttataagggattttgccgatttcggcctattggttaaaaaatgagctgatttaacaaaaatttaacgcgaattttaacaaaatattaacgcttacaatttaggtggcacttttcggggaaatgtgcgcggaacccctatttgtttatttttctaaatacattcaaatatgtatccgctcatgagacaataaccctgataaatgcttcaataatattgaaaaaggaagagtatgattgaacaagatggattgcacgcaggttctccggccgcttgggtggagaggctattcggctatgactgggcacaacagacaatcggctgctctgatgccgccgtgttccggctgtcagcgcaggggcgcccggttctttttgtcaagaccgacctgtccggtgccctgaatgaactgcaagacgaggcagcgcggctatcgtggctggccacgacgggcgttccttgcgcagctgtgctcgacgttgtcactgaagcgggaagggactggctgctattgggcgaagtgccggggcaggatctcctgtcatctcaccttgctcctgccgagaaagtatccatcatggctgatgcaatgcggcggctgcatacgcttgatccggctacctgcccattcgaccaccaagcgaaacatcgcatcgagcgagcacgtactcggatggaagccggtcttgtcgatcaggatgatctggacgaagagcatcaggggctcgcgccagccgaactgttcgccaggctcaaggcgagcatgcccgacggcgaggatctcgtcgtgacccatggcgatgcctgcttgccgaatatcatggtggaaaatggccgcttttctggattcatcgactgtggccggctgggtgtggcggaccgctatcaggacatagcgttggctacccgtgatattgctgaagagcttggcggcgaatgggctgaccgcttcctcgtgctttacggtatcgccgctcccgattcgcagcgcatcgccttctatcgccttcttgacgagttcttctgactgtcagaccaagtttactcatatatactttagattgatttaaaacttcatttttaatttaaaaggatctaggtgaagatcctttttgataatctcatgaccaaaatcccttaacgtgagttttcgttccactgagcgtcagaccccgtagaaaagatcaaaggatcttcttgagatcctttttttctgcgcgtaatctgctgcttgcaaacaaaaaaaccaccgctaccagcggtggtttgtttgccggatcaagagctaccaactctttttccgaaggtaactggcttcagcagagcgcagataccaaatactgttcttctagtgtagccgtagttaggccaccacttcaagaactctgtagcaccgcctacatacctcgctctgctaatcctgttaccagtggctgctgccagtggcgataagtcgtgtcttaccgggttggactcaagacgatagttaccggataaggcgcagcggtcgggctgaacggggggttcgtgcacacagcccagcttggagcgaacgacctacaccgaactgagatacctacagcgtgagctatgagaaagcgccacgcttcccgaagggagaaaggcggacaggtatccggtaagcggcagggtcggaacaggagagcgcacgagggagcttccagggggaaacgcctggtatctttatagtcctgtcgggtttcgccacctctgacttgagcgtcgatttttgtgatgctcgtcaggggggcggagcctatggaaaaacgccagcaacgcggcctttttacggttcctggccttttgctggccttttgctcacatgttctttcctgcgttatcccctgattctgtggataaccgtattaccgcctttgagtgagctgataccgctcgccgcagccgaacgaccgagcgcagcgagtcagtgagcgaggaagcggaagagcgcccaatacgcaaaccgcctctccccgcgcgttggccgattcattaatgcagctggcacgacaggtttcccgactggaaagcgggcagtgagcgcaacgcaattaatgtgagttagctcactcattaggcaccccaggctttacactttatgcttccggctcgtatgttgtgtggaattgtgagcggataacaatttcacacaggaaacagctatgaccatgattacgccagatttaattaaggccttaattaggctgcgcgctcgctcgctcactgaggccgcccgggcaaagcccgggcgtcgggcgacctttggtcgcccggcctcagtgagcgagcgagcgcgcagagagggagtggccaactccatcactaggggttccttgtagttaatgattaacccgccatgctacttatctaccagggtaatggggatcctctagaactatagctagtcgacattgattattgactagttattaatagtaatcaattacggggtcattagttcatagcccatatatggagttccgcgttacataacttacggtaaatggcccgcctggctgaccgcccaacgacccccgcccattgacgtcaataatgacgtatgttcccatagtaacgccaatagggactttccattgacgtcaatgggtggagtatttacggtaaactgcccacttggcagtacatcaagtgtatcatatgccaagtacgccccctattgacgtcaatgacggtaaatggcccgcctggcattatgcccagtacatgaccttatgggactttcctacttggcagtacatctacgtattagtcatcgctattaccatggtcgaggtgagccccacgttctgcttcactctccccatctcccccccctccccacccccaattttgtatttatttattttttaattattttgtgcagcgatgggggcggggggggggggggggcgcgcgccaggcggggcggggcggggcgaggggcggggcggggcaaggcggagaggtgcggcggcagccaatcagagcggcgcgctccgaaagtttccttttatggcgaggcggcggcggcggcggccctataaaaagcgaagcgcgcggcgggcgggagtcgctgcgcgctgccttcgccccgtgccccgctccgccgccgcctcgcgccgcccgccccggctctgactgaccgcgttactcccacaggtgagcgggcgggacggcccttctcctccgggctgtaattagcgcttggtttaatgacggcttgtttcttttctgtggctgcgtgaaagccttgaggggctccgggagggccctttgtgcggggggagcggctcggggggtgcgtgcgtgtgtgtgtgcgtggggagcgccgcgtgcggctccgcgctgcccggcggctgtgagcgctgcgggcgcggcgcggggctttgtgcgctccgcagtgtgcgcgaggggagcgcggccgggggcggtgccccgcggtgcggggggggctgcgaggggaacaaaggctgcgtgcggggtgtgtgcgtgggggggtgagcagggggtgtgggcgcgtcggtcgggctgcaaccccccctgcacccccctccccgagttgctgagcacggcccggcttcgggtgcggggctccgtacggggcgtggcgcggggctcgccgtgccgggcggggggtggcggcaggtgggggtgccgggcggggcggggccgcctcgggccggggagggctcgggggaggggcgcggcggcccccggagcgccggcggctgtcgaggcgcggcgagccgcagccattgccttttatggtaatcgtgcgagagggcgcagggacttcctttgtcccaaatctgtgcggagccgaaatctgggaggcgccgccgcaccccctctagcgggcgcggggcgaagcggtgcggcgccggcaggaaggaaatgggcggggagggccttcgtgcgtcgccgcgccgccgtccccttctccctctccagcctcggggctgtccgcggggggacggctgccttcgggggggacggggcagggcggggttcggcttctggcgtgtgaccggcggctctagagcctctgctaaccatgttcatgccttcttctttttcctacagctcctgggcaacgtgctggttattgtgctgtctcatcattttggcaaagaattcgccgccaccatggtgtcctattgggatacaggagtgctgctgtgtgctctgctgagctgtctgctgctgacaggctcttcttcaggctctgacacaggcagaccctttgtggagatgtactctgaaatccctgagatcattcacatgacagaaggcagagaactggtgattccctgcagggttaccagcccaaacatcacagtgaccctgaagaagttccccctggacaccctgatccctgatggcaaaagaatcatctgggactctaggaaaggctttatcatctccaatgccacatacaaagagattggcctgctgacctgtgaggctactgtcaatggccacctgtacaaaacaaattacctgacccacagacagaccaacacaatcattgatgtggtgctgagcccatcccatggcattgagctgtctgtgggagaaaagctggtgctgaattgtacagctagaacagaacttaatgtgggcattgatttcaactgggagtaccctagctccaagcaccagcataaaaagctggtgaacagagacctgaagacccagtctggctctgagatgaaaaagttcttgagcaccctgaccattgatggagtgaccagatctgaccagggcctgtacacctgtgctgcctcctctgggctgatgacaaaaaagaacagcacctttgtgagagtgcatgagaaggataaaacccacacctgccctccttgtcctgctcctgagctgctggggggaccatctgtgttcctgttcccccccaagcccaaggataccctgatgatcagcagaaccccagaagtgacctgtgtggtggtggatgtgtcccatgaggacccagaggtgaaattcaactggtatgtggatggagtggaggtgcacaatgccaagaccaaaccaagagaggagcagtataactccacctacagggtggtgtctgtgctgactgtgctgcaccaggattggctgaatggcaaggagtacaagtgcaaggttagcaataaagctctgcctgcccccattgaaaagaccatttccaaagccaaagggcagccaagggagccccaggtgtacaccctgcccccatctagagatgagctgaccaagaaccaggtgagcctcacatgtctggtgaagggcttttacccttctgacattgctgtggagtgggaaagcaatggacagcctgagaataactataagaccacacccccagtgctggattctgatggcagttttttcctgtactctaagctgacagtggacaaatccagatggcagcagggcaatgtgttcagctgctctgtgatgcatgaggccctgcacaatcactatacacagaagagcctgagcctgagcccagggaagtga

SEQ ID NO: 31 - DNA, 3781 bp, synthetic construct
  source 1..3781: mol_type = other DNA
ctgcgcgctcgctcgctcactgaggccgcccgggcaaagcccgggcgtcgggcgacctttggtcgcccggcctcagtgagcgagcgagcgcgcagagagggagtggccaactccatcactaggggttccttgtagttaatgattaacccgccatgctacttatctaccagggtaatggggatcctctagaactatagctagtcgacattgattattgactagttattaatagtaatcaattacggggtcattagttcatagcccatatatggagttccgcgttacataacttacggtaaatggcccgcctggctgaccgcccaacgacccccgcccattgacgtcaataatgacgtatgttcccatagtaacgccaatagggactttccattgacgtcaatgggtggagtatttacggtaaactgcccacttggcagtacatcaagtgtatcatatgccaagtacgccccctattgacgtcaatgacggtaaatggcccgcctggcattatgcccagtacatgaccttatgggactttcctacttggcagtacatctacgtattagtcatcgctattaccatggtcgaggtgagccccacgttctgcttcactctccccatctcccccccctccccacccccaattttgtatttatttattttttaattattttgtgcagcgatgggggcggggggggggggggggcgcgcgccaggcggggcggggcggggcgaggggcggggcggggcgaggcggagaggtgcggcggcagccaatcagagcggcgcgctccgaaagtttccttttatggcgaggcggcggcggcggcggccctataaaaagcgaagcgcgcggcgggcggggagtcgctgcgacgctgccttcgccccgtgccccgctccgccgccgcctcgcgccgcccgccccggctctgactgaccgcgttactcccacaggtgagcgggcgggacggcccttctcctccgggctgtaattagcgcttggtttaatgacggcttgtttcttttctgtggctgcgtgaaagccttgaggggctccgggagggccctttgtgcggggggagcggctcggggggtgcgtgcgtgtgtgtgtgcgtggggagcgccgcgtgcggctccgcgctgcccggcggctgtgagcgctgcgggcgcggcgcggggctttgtgcgctccgcagtgtgcgcgaggggagcgcggccgggggcggtgccccgcggtgcggggggggctgcgaggggaacaaaggctgcgtgcggggtgtgtgcgtgggggggtgagcagggggtgtgggcgcgtcggtcgggctgcaaccccccctgcacccccctccccgagttgctgagcacggcccggcttcgggtgcggggctccgtacggggcgtggcgcggggctcgccgtgccgggcggggggtggcggcaggtgggggtgccgggcggggcggggccgcctcgggccggggagggctcgggggaggggcgcggcggcccccggagcgccggcggctgtcgaggcgcggcgagccgcagccattgccttttatggtaatcgtgcgagagggcgcagggacttcctttgtcccaaatctgtgcggagccgaaatctgggaggcgccgccgcaccccctctagcgggcgcggggcgaagcggtgcggcgccggcaggaaggaaatgggcggggagggccttcgtgcgtcgccgcgccgccgtccccttctccctctccagcctcggggctgtccgcggggggacggctgccttcgggggggacggggcagggcggggttcggcttctggcgtgtgaccggcggctctagagcctctgctaaccatgttcatgccttcttctttttcctacagctcctgggcaacgtgctggttattgtgctgtctcatcattttggcaaagaattcgccgccaccatggtgtcctattgggatacaggagtgctgctgtgtgctctgctgagctgtctgctgctgacaggctcttcttcaggctctgacacaggcagaccctttgtggagatgtactctgaaatccctgagatcattcacatgacagaaggcagagaactggtgattccctgcagggttaccagcccaaacatcacagtgaccctgaagaagttccccctggacaccctgatccctgatggcaaaagaatcatctgggactctaggtgagtatctcagggatccagacatggggatatgggaggtgcctctgatcccagggctcactgtgggtctctctgttcacaggaaaggctttatcatctccaatgccacatacaaagagattggcctgctgacctgtgaggctactgtcaatggccacctgtacaaaacaaattacctgacccacagacagaccaacacaatcattgatgtggtgctgagcccatcccatggcattgagctgtctgtgggagaaaagctggtgctgaattgtacagctagaacagaacttaatgtgggcattgatttcaactgggagtaccctagctccaagcaccagcataaaaagctggtgaacagagacctgaagacccagtctggctctgagatgaaaaagttcttgagcaccctgaccattgatggagtgaccagatctgaccagggcctgtacacctgtgctgcctcctctgggctgatgacaaaaaagaacagcacctttgtgagagtgcatgagaaggataaaacccacacctgccctccttgtcctgctcctgagctgctggggggaccatctgtgttcctgttcccccccaagcccaaggataccctgatgatcagcagaaccccagaagtgacctgtgtggtggtggatgtgtcccatgaggacccagaggtgaaattcaactggtatgtggatggagtggaggtgcacaatgccaagaccaaaccaagagaggagcagtataactccacctacagggtggtgtctgtgctgactgtgctgcaccaggattggctgaatggcaaggagtacaagtgcaaggttagcaataaagctctgcctgcccccattgaaaagaccatttccaaagccaaagggcagccaagggagccccaggtgtacaccctgcccccatctagagatgagctgaccaagaaccaggtgagcctcacatgtctggtgaagggcttttacccttctgacattgctgtggagtgggaaagcaatggacagcctgagaataactataagaccacacccccagtgctggattctgatggcagttttttcctgtactctaagctgacagtggacaaatccagatggcagcagggcaatgtgttcagctgctctgtgatgcatgaggccctgcacaatcactatacacagaagagcctgagcctgagcccagggaagtgactcgaggacggggtgaactacgcctgaggatccgatctttttccctctgccaaaaattatggggacatcatgaagccccttgagcatctgacttctggctaataaaggaaatttattttcattgcaatagtgtgttggaattttttgtgtctctcactcggaagcaattcgttgatctgaatttcgaccacccataatacccattaccctggtagataagtagcatggcgggttaatcattaactacaaggaacccctagtgatggagttggccactccctctctgcgcgctcgctcgctcactgaggccgggcgaccaaaggtcgcccgacgcccgggctttgcccgggcggcctcagtgagcgagcgagcgcgcag

SEQ ID NO: 32 - DNA, 6536 bp, synthetic construct
  source 1..6536: mol_type = other DNA
ctcgaggacggggtgaactacgcctgaggatccgatctttttccctctgccaaaaattatggggacatcatgaagccccttgagcatctgacttctggctaataaaggaaatttattttcattgcaatagtgtgttggaattttttgtgtctctcactcggaagcaattcgttgatctgaatttcgaccacccataatacccattaccctggtagataagtagcatggcgggttaatcattaactacaaggaacccctagtgatggagttggccactccctctctgcgcgctcgctcgctcactgaggccgggcgaccaaaggtcgcccgacgcccgggctttgcccgggcggcctcagtgagcgagcgagcgcgcagccttaattaacctaattcactggccgtcgttttacaacgtcgtgactgggaaaaccctggcgttacccaacttaatcgccttgcagcacatccccctttcgccagctggcgtaatagcgaagaggcccgcaccgatcgcccttcccaacagttgcgcagcctgaatggcgaatgggacgcgccctgtagcggcgcattaagcgcggcgggtgtggtggttacgcgcagcgtgaccgctacacttgccagcgccctagcgcccgctcctttcgctttcttcccttcctttctcgccacgttcgccggctttccccgtcaagctctaaatcgggggctccctttagggttccgatttagtgctttacggcacctcgaccccaaaaaacttgattagggtgatggttcacgtagtgggccatcgccctgatagacggtttttcgccctttgacgttggagtccacgttctttaatagtggactcttgttccaaactggaacaacactcaaccctatctcggtctattcttttgatttataagggattttgccgatttcggcctattggttaaaaaatgagctgatttaacaaaaatttaacgcgaattttaacaaaatattaacgcttacaatttaggtggcacttttcggggaaatgtgcgcggaacccctatttgtttatttttctaaatacattcaaatatgtatccgctcatgagacaataaccctgataaatgcttcaataatattgaaaaaggaagagtatgattgaacaagatggattgcacgcaggttctccggccgcttgggtggagaggctattcggctatgactgggcacaacagacaatcggctgctctgatgccgccgtgttccggctgtcagcgcaggggcgcccggttctttttgtcaagaccgacctgtccggtgccctgaatgaactgcaagacgaggcagcgcggctatcgtggctggccacgacgggcgttccttgcgcagctgtgctcgacgttgtcactgaagcgggaagggactggctgctattgggcgaagtgccggggcaggatctcctgtcatctcaccttgctcctgccgagaaagtatccatcatggctgatgcaatgcggcggctgcatacgcttgatccggctacctgcccattcgaccaccaagcgaaacatcgcatcgagcgagcacgtactcggatggaagccggtcttgtcgatcaggatgatctggacgaagagcatcaggggctcgcgccagccgaactgttcgccaggctcaaggcgagcatgcccgacggcgaggatctcgtcgtgacccatggcgatgcctgcttgccgaatatcatggtggaaaatggccgcttttctggattcatcgactgtggccggctgggtgtggcggaccgctatcaggacatagcgttggctacccgtgatattgctgaagagcttggcggcgaatgggctgaccgcttcctcgtgctttacggtatcgccgctcccgattcgcagcgcatcgccttctatcgccttcttgacgagttcttctgactgtcagaccaagtttactcatatatactttagattgatttaaaacttcatttttaatttaaaaggatctaggtgaagatcctttttgataatctcatgaccaaaatcccttaacgtgagttttcgttccactgagcgtcagaccccgtagaaaagatcaaaggatcttcttgagatcctttttttctgcgcgtaatctgctgcttgcaaacaaaaaaaccaccgctaccagcggtggtttgtttgccggatcaagagctaccaactctttttccgaaggtaactggcttcagcagagcgcagataccaaatactgttcttctagtgtagccgtagttaggccaccacttcaagaactctgtagcaccgcctacatacctcgctctgctaatcctgttaccagtggctgctgccagtggcgataagtcgtgtcttaccgggttggactcaagacgatagttaccggataaggcgcagcggtcgggctgaacggggggttcgtgcacacagcccagcttggagcgaacgacctacaccgaactgagatacctacagcgtgagctatgagaaagcgccacgcttcccgaagggagaaaggcggacaggtatccggtaagcggcagggtcggaacaggagagcgcacgagggagcttccagggggaaacgcctggtatctttatagtcctgtcgggtttcgccacctctgacttgagcgtcgatttttgtgatgctcgtcaggggggcggagcctatggaaaaacgccagcaacgcggcctttttacggttcctggccttttgctggccttttgctcacatgttctttcctgcgttatcccctgattctgtggataaccgtattaccgcctttgagtgagctgataccgctcgccgcagccgaacgaccgagcgcagcgagtcagtgagcgaggaagcggaagagcgcccaatacgcaaaccgcctctccccgcgcgttggccgattcattaatgcagctggcacgacaggtttcccgactggaaagcgggcagtgagcgcaacgcaattaatgtgagttagctcactcattaggcaccccaggctttacactttatgcttccggctcgtatgttgtgtggaattgtgagcggataacaatttcacacaggaaacagctatgaccatgattacgccagatttaattaaggccttaattaggctgcgcgctcgctcgctcactgaggccgcccgggcaaagcccgggcgtcgggcgacctttggtcgcccggcctcagtgagcgagcgagcgcgcagagagggagtggccaactccatcactaggggttccttgtagttaatgattaacccgccatgctacttatctaccagggtaatggggatcctctagaactatagctagtcgacattgattattgactagttattaatagtaatcaattacggggtcattagttcatagcccatatatggagttccgcgttacataacttacggtaaatggcccgcctggctgaccgcccaacgacccccgcccattgacgtcaataatgacgtatgttcccatagtaacgccaatagggactttccattgacgtcaatgggtggagtatttacggtaaactgcccacttggcagtacatcaagtgtatcatatgccaagtacgccccctattgacgtcaatgacggtaaatggcccgcctggcattatgcccagtacatgaccttatgggactttcctacttggcagtacatctacgtattagtcatcgctattaccatggtcgaggtgagccccacgttctgcttcactctccccatctcccccccctccccacccccaattttgtatttatttattttttaattattttgtgcagcgatgggggcggggggggggggggggcgcgcgccaggcggggcggggcggggcgaggggcggggcggggcgaggcggagaggtgcggcggcagccaatcagagcggcgcgctccgaaagtttccttttatggcgaggcggcggcggcggcggccctataaaaagcgaagcgcgcggcgggcggggagtcgctgcgacgctgccttcgccccgtgccccgctccgccgccgcctcgcgccgcccgccccggctctgactgaccgcgttactcccacaggtgagcgggcgggacggcccttctcctccgggctgtaattagcgcttggtttaatgacggcttgtttcttttctgtggctgcgtgaaagccttgaggggctccgggagggccctttgtgcggggggagcggctcggggggtgcgtgcgtgtgtgtgtgcgtggggagcgccgcgtgcggctccgcgctgcccggcggctgtgagcgctgcgggcgcggcgcggggctttgtgcgctccgcagtgtgcgcgaggggagcgcggccgggggcggtgccccgcggtgcggggggggctgcgaggggaacaaaggctgcgtgcggggtgtgtgcgtgggggggtgagcagggggtgtgggcgcgtcggtcgggctgcaaccccccctgcacccccctccccgagttgctgagcacggcccggcttcgggtgcggggctccgtacggggcgtggcgcggggctcgccgtgccgggcggggggtggcggcaggtgggggtgccgggcggggcggggccgcctcgggccggggagggctcgggggaggggcgcggcggcccccggagcgccggcggctgtcgaggcgcggcgagccgcagccattgccttttatggtaatcgtgcgagagggcgcagggacttcctttgtcccaaatctgtgcggagccgaaatctgggaggcgccgccgcaccccctctagcgggcgcggggcgaagcggtgcggcgccggcaggaaggaaatgggcggggagggccttcgtgcgtcgccgcgccgccgtccccttctccctctccagcctcggggctgtccgcggggggacggctgccttcgggggggacggggcagggcggggttcggcttctggcgtgtgaccggcggctctagagcctctgctaaccatgttcatgccttcttctttttcctacagctcctgggcaacgtgctggttattgtgctgtctcatcattttggcaaagaattcgccgccaccatggtgtcctattgggatacaggagtgctgctgtgtgctctgctgagctgtctgctgctgacaggctcttcttcaggctctgacacaggcagaccctttgtggagatgtactctgaaatccctgagatcattcacatgacagaaggcagagaactggtgattccctgcagggttaccagcccaaacatcacagtgaccctgaagaagttccccctggacaccctgatccctgatggcaaaagaatcatctgggactctaggtgagtatctcagggatccagacatggggatatgggaggtgcctctgatcccagggctcactgtgggtctctctgttcacaggaaaggctttatcatctccaatgccacatacaaagagattggcctgctgacctgtgaggctactgtcaatggccacctgtacaaaacaaattacctgacccacagacagaccaacacaatcattgatgtggtgctgagcccatcccatggcattgagctgtctgtgggagaaaagctggtgctgaattgtacagctagaacagaacttaatgtgggcattgatttcaactgggagtaccctagctccaagcaccagcataaaaagctggtgaacagagacctgaagacccagtctggctctgagatgaaaaagttcttgagcaccctgaccattgatggagtgaccagatctgaccagggcctgtacacctgtgctgcctcctctgggctgatgacaaaaaagaacagcacctttgtgagagtgcatgagaaggataaaacccacacctgccctccttgtcctgctcctgagctgctggggggaccatctgtgttcctgttcccccccaagcccaaggataccctgatgatcagcagaaccccagaagtgacctgtgtggtggtggatgtgtcccatgaggacccagaggtgaaattcaactggtatgtggatggagtggaggtgcacaatgccaagaccaaaccaagagaggagcagtataactccacctacagggtggtgtctgtgctgactgtgctgcaccaggattggctgaatggcaaggagtacaagtgcaaggttagcaataaagctctgcctgcccccattgaaaagaccatttccaaagccaaagggcagccaagggagccccaggtgtacaccctgcccccatctagagatgagctgaccaagaaccaggtgagcctcacatgtctggtgaagggcttttacccttctgacattgctgtggagtgggaaagcaatggacagcctgagaataactataagaccacacccccagtgctggattctgatggcagttttttcctgtactctaagctgacagtggacaaatccagatggcagcagggcaatgtgttcagctgctctgtgatgcatgaggccctgcacaatcactatacacagaagagcctgagcctgagcccagggaagtga

SEQ ID NO: 33 - DNA, 3874 bp, synthetic construct
  source 1..3874: mol_type = other DNA
ctgcgcgctcgctcgctcactgaggccgcccgggcaaagcccgggcgtcgggcgacctttggtcgcccggcctcagtgagcgagcgagcgcgcagagagggagtggccaactccatcactaggggttccttgtagttaatgattaacccgccatgctacttatctaccagggtaatggggatcctctagaactatagctagtcgacattgattattgactagttattaatagtaatcaattacggggtcattagttcatagcccatatatggagttccgcgttacataacttacggtaaatggcccgcctggctgaccgcccaacgacccccgcccattgacgtcaataatgacgtatgttcccatagtaacgccaatagggactttccattgacgtcaatgggtggagtatttacggtaaactgcccacttggcagtacatcaagtgtatcatatgccaagtacgccccctattgacgtcaatgacggtaaatggcccgcctggcattatgcccagtacatgaccttatgggactttcctacttggcagtacatctacgtattagtcatcgctattaccatggtcgaggtgagccccacgttctgcttcactctccccatctcccccccctccccacccccaattttgtatttatttattttttaattattttgtgcagcgatgggggcggggggggggggggggcgcgcgccaggcggggcggggcggggcgaggggcggggcggggcaaggcggagaggtgcggcggcagccaatcagagcggcgcgctccgaaagtttccttttatggcgaggcggcggcggcggcggccctataaaaagcgaagcgcgcggcgggcgggagtcgctgcgcgctgccttcgccccgtgccccgctccgccgccgcctcgcgccgcccgccccggctctgactgaccgcgttactcccacaggtgagcgggcgggacggcccttctcctccgggctgtaattagcgcttggtttaatgacggcttgtttcttttctgtggctgcgtgaaagccttgaggggctccgggagggccctttgtgcggggggagcggctcggggggtgcgtgcgtgtgtgtgtgcgtggggagcgccgcgtgcggctccgcgctgcccggcggctgtgagcgctgcgggcgcggcgcggggctttgtgcgctccgcagtgtgcgcgaggggagcgcggccgggggcggtgccccgcggtgcggggggggctgcgaggggaacaaaggctgcgtgcggggtgtgtgcgtgggggggtgagcagggggtgtgggcgcgtcggtcgggctgcaaccccccctgcacccccctccccgagttgctgagcacggcccggcttcgggtgcggggctccgtacggggcgtggcgcggggctcgccgtgccgggcggggggtggcggcaggtgggggtgccgggcggggcggggccgcctcgggccggggagggctcgggggaggggcgcggcggcccccggagcgccggcggctgtcgaggcgcggcgagccgcagccattgccttttatggtaatcgtgcgagagggcgcagggacttcctttgtcccaaatctgtgcggagccgaaatctgggaggcgccgccgcaccccctctagcgggcgcggggcgaagcggtgcggcgccggcaggaaggaaatgggcggggagggccttcgtgcgtcgccgcgccgccgtccccttctccctctccagcctcggggctgtccgcggggggacggctgccttcgggggggacggggcagggcggggttcggcttctggcgtgtgaccggcggctctagagcctctgctaaccatgttcatgccttcttctttttcctacagctcctgggcaacgtgctggttattgtgctgtctcatcattttggcaaagaattcgccgccaccatggtgtcctattgggatacaggagtgctgctgtgtgctctgctgagctgtctgctgctgacaggctcttcttcaggcaggtgagtatctcagggatccagacatggggatatgggaggtgcctctgatcccagggctcactgtgggtctctctgttcacagggacacaggcagaccctttgtggagatgtactctgaaatccctgagatcattcacatgacagaaggcagagaactggtgattccctgcagggttaccagcccaaacatcacagtgaccctgaagaagttccccctggacaccctgatccctgatggcaaaagaatcatctgggactctaggaaaggctttatcatctccaatgccacatacaaagagattggcctgctgacctgtgaggctactgtcaatggccacctgtacaaaacaaattacctgacccacagacagaccaacacaatcattgatgtggtgctgagcccatcccatggcattgagctgtctgtgggagaaaagctggtgctgaattgtacagctagaacagaacttaatgtgggcattgatttcaactgggagtaccctagctccaagcaccagcataaaaagctggtgaacagagacctgaagacccagtctggctctgagatgaaaaagttcttgagcaccctgaccattgatggagtgaccagatctgaccagggcctgtacacctgtgctgcctcctctgggctgatgacaaaaaagaacagcacctttgtgagagtgcatgagaaggataaaacccacacctgccctccttgtcctgctcctgagctgctggggggaccatctgtgttcctgttcccccccaagcccaaggataccctgatgatcagcagaaccccagaagtgacctgtgtggtggtggatgtgtcccatgaggacccagaggtgaaattcaactggtatgtggatggagtggaggtgcacaatgccaagaccaaaccaagagaggagcagtataactccacctacagggtggtgtctgtgctgactgtgctgcaccaggattggctgaatggcaaggagtacaagtgcaaggttagcaataaagctctgcctgcccccattgaaaagaccatttccaaagccaaagggcagccaagggagccccaggtgtacaccctgcccccatctagagatgagctgaccaagaaccaggtgagcctcacatgtctggtgaagggcttttacccttctgacattgctgtggagtgggaaagcaatggacagcctgagaataactataagaccacacccccagtgctggattctgatggcagttttttcctgtactctaagctgacagtggacaaatccagatggcagcagggcaatgtgttcagctgctctgtgatgcatgaggccctgcacaatcactatacacagaagagcctgagcctgagcccagggaagtgactcgaggacggggtgaactacgcctgaggatcccagacatgataagatacattgatgagtttggacaaaccacaactagaatgcagtgaaaaaaatgctttatttgtgaaatttgtgatgctattgctttatttgtaaccattataagctgcaataaacaagttaacaacaacaattgcattcattttatgtttcaggttcagggggagatgtgggaggttttttaaagcaagtaaaacctctacaaatgtggtagaagcaattcgttgatctgaatttcgaccacccataatacccattaccctggtagataagtagcatggcgggttaatcattaactacaaggaacccctagtgatggagttggccactccctctctgcgcgctcgctcgctcactgaggccgggcgaccaaaggtcgcccgacgcccgggctttgcccgggcggcctcagtgagcgagcgagcgcgcag

SEQ ID NO: 34 - DNA, 6629 bp, synthetic construct
  source 1..6629: mol_type = other DNA
ctcgaggacggggtgaactacgcctgaggatcccagacatgataagatacattgatgagtttggacaaaccacaactagaatgcagtgaaaaaaatgctttatttgtgaaatttgtgatgctattgctttatttgtaaccattataagctgcaataaacaagttaacaacaacaattgcattcattttatgtttcaggttcagggggagatgtgggaggttttttaaagcaagtaaaacctctacaaatgtggtagaagcaattcgttgatctgaatttcgaccacccataatacccattaccctggtagataagtagcatggcgggttaatcattaactacaaggaacccctagtgatggagttggccactccctctctgcgcgctcgctcgctcactgaggccgggcgaccaaaggtcgcccgacgcccgggctttgcccgggcggcctcagtgagcgagcgagcgcgcagccttaattaacctaattcactggccgtcgttttacaacgtcgtgactgggaaaaccctggcgttacccaacttaatcgccttgcagcacatccccctttcgccagctggcgtaatagcgaagaggcccgcaccgatcgcccttcccaacagttgcgcagcctgaatggcgaatgggacgcgccctgtagcggcgcattaagcgcggcgggtgtggtggttacgcgcagcgtgaccgctacacttgccagcgccctagcgcccgctcctttcgctttcttcccttcctttctcgccacgttcgccggctttccccgtcaagctctaaatcgggggctccctttagggttccgatttagtgctttacggcacctcgaccccaaaaaacttgattagggtgatggttcacgtagtgggccatcgccctgatagacggtttttcgccctttgacgttggagtccacgttctttaatagtggactcttgttccaaactggaacaacactcaaccctatctcggtctattcttttgatttataagggattttgccgatttcggcctattggttaaaaaatgagctgatttaacaaaaatttaacgcgaattttaacaaaatattaacgcttacaatttaggtggcacttttcggggaaatgtgcgcggaacccctatttgtttatttttctaaatacattcaaatatgtatccgctcatgagacaataaccctgataaatgcttcaataatattgaaaaaggaagagtatgattgaacaagatggattgcacgcaggttctccggccgcttgggtggagaggctattcggctatgactgggcacaacagacaatcggctgctctgatgccgccgtgttccggctgtcagcgcaggggcgcccggttctttttgtcaagaccgacctgtccggtgccctgaatgaactgcaagacgaggcagcgcggctatcgtggctggccacgacgggcgttccttgcgcagctgtgctcgacgttgtcactgaagcgggaagggactggctgctattgggcgaagtgccggggcaggatctcctgtcatctcaccttgctcctgccgagaaagtatccatcatggctgatgcaatgcggcggctgcatacgcttgatccggctacctgcccattcgaccaccaagcgaaacatcgcatcgagcgagcacgtactcggatggaagccggtcttgtcgatcaggatgatctggacgaagagcatcaggggctcgcgccagccgaactgttcgccaggctcaaggcgagcatgcccgacggcgaggatctcgtcgtgacccatggcgatgcctgcttgccgaatatcatggtggaaaatggccgcttttctggattcatcgactgtggccggctgggtgtggcggaccgctatcaggacatagcgttggctacccgtgatattgctgaagagcttggcggcgaatgggctgaccgcttcctcgtgctttacggtatcgccgctcccgattcgcagcgcatcgccttctatcgccttcttgacgagttcttctgactgtcagaccaagtttactcatatatactttagattgatttaaaacttcatttttaatttaaaaggatctaggtgaagatcctttttgataatctcatgaccaaaatcccttaacgtgagttttcgttccactgagcgtcagaccccgtagaaaagatcaaaggatcttcttgagatcctttttttctgcgcgtaatctgctgcttgcaaacaaaaaaaccaccgctaccagcggtggtttgtttgccggatcaagagctaccaactctttttccgaaggtaactggcttcagcagagcgcagataccaaatactgttcttctagtgtagccgtagttaggccaccacttcaagaactctgtagcaccgcctacatacctcgctctgctaatcctgttaccagtggctgctgccagtggcgataagtcgtgtcttaccgggttggactcaagacgatagttaccggataaggcgcagcggtcgggctgaacggggggttcgtgcacacagcccagcttggagcgaacgacctacaccgaactgagatacctacagcgtgagctatgagaaagcgccacgcttcccgaagggagaaaggcggacaggtatccggtaagcggcagggtcggaacaggagagcgcacgagggagcttccagggggaaacgcctggtatctttatagtcctgtcgggtttcgccacctctgacttgagcgtcgatttttgtgatgctcgtcaggggggcggagcctatggaaaaacgccagcaacgcggcctttttacggttcctggccttttgctggccttttgctcacatgttctttcctgcgttatcccctgattctgtggataaccgtattaccgcctttgagtgagctgataccgctcgccgcagccgaacgaccgagcgcagcgagtcagtgagcgaggaagcggaagagcgcccaatacgcaaaccgcctctccccgcgcgttggccgattcattaatgcagctggcacgacaggtttcccgactggaaagcgggcagtgagcgcaacgcaattaatgtgagttagctcactcattaggcaccccaggctttacactttatgcttccggctcgtatgttgtgtggaattgtgagcggataacaatttcacacaggaaacagctatgaccatgattacgccagatttaattaaggccttaattaggctgcgcgctcgctcgctcactgaggccgcccgggcaaagcccgggcgtcgggcgacctttggtcgcccggcctcagtgagcgagcgagcgcgcagagagggagtggccaactccatcactaggggttccttgtagttaatgattaacccgccatgctacttatctaccagggtaatggggatcctctagaactatagctagtcgacattgattattgactagttattaatagtaatcaattacggggtcattagttcatagcccatatatggagttccgcgttacataacttacggtaaatggcccgcctggctgaccgcccaacgacccccgcccattgacgtcaataatgacgtatgttcccatagtaacgccaatagggactttccattgacgtcaatgggtggagtatttacggtaaactgcccacttggcagtacatcaagtgtatcatatgccaagtacgccccctattgacgtcaatgacggtaaatggcccgcctggcattatgcccagtacatgaccttatgggactttcctacttggcagtacatctacgtattagtcatcgctattaccatggtcgaggtgagccccacgttctgcttcactctccccatctcccccccctccccacccccaattttgtatttatttattttttaattattttgtgcagcgatgggggcggggggggggggggggcgcgcgccaggcggggcggggcggggcgaggggcggggcggggcgaggcggagaggtgcggcggcagccaatcagagcggcgcgctccgaaagtttccttttatggcgaggcggcggcggcggcggccctataaaaagcgaagcgcgcggcgggcgggagtcgctgcgcgctgccttcgccccgtgccccgctccgccgccgcctcgcgccgcccgccccggctctgactgaccgcgttactcccacaggtgagcgggcgggacggcccttctcctccgggctgtaattagcgcttggtttaatgacggcttgtttcttttctgtggctgcgtgaaagccttgaggggctccgggagggccctttgtgcggggggagcggctcggggggtgcgtgcgtgtgtgtgtgcgtggggagcgccgcgtgcggctccgcgctgcccggcggctgtgagcgctgcgggcgcggcgcggggctttgtgcgctccgcagtgtgcgcgaggggagcgcggccgggggcggtgccccgcggtgcggggggggctgcgaggggaacaaaggctgcgtgcggggtgtgtgcgtgggggggtgagcagggggtgtgggcgcgtcggtcgggctgcaaccccccctgcacccccctccccgagttgctgagcacggcccggcttcgggtgcggggctccgtacggggcgtggcgcggggctcgccgtgccgggcggggggtggcggcaggtgggggtgccgggcggggcggggccgcctcgggccggggagggctcgggggaggggcgcggcggcccccggagcgccggcggctgtcgaggcgcggcgagccgcagccattgccttttatggtaatcgtgcgagagggcgcagggacttcctttgtcccaaatctgtgcggagccgaaatctgggaggcgccgccgcaccccctctagcgggcgcggggcgaagcggtgcggcgccggcaggaaggaaatgggcggggagggccttcgtgcgtcgccgcgccgccgtccccttctccctctccagcctcggggctgtccgcggggggacggctgccttcgggggggacggggcagggcggggttcggcttctggcgtgtgaccggcggctctagagcctctgctaaccatgttcatgccttcttctttttcctacagctcctgggcaacgtgctggttattgtgctgtctcatcattttggcaaagaattcgccgccaccatggtgtcctattgggatacaggagtgctgctgtgtgctctgctgagctgtctgctgctgacaggctcttcttcaggcaggtgagtatctcagggatccagacatggggatatgggaggtgcctctgatcccagggctcactgtgggtctctctgttcacagggacacaggcagaccctttgtggagatgtactctgaaatccctgagatcattcacatgacagaaggcagagaactggtgattccctgcagggttaccagcccaaacatcacagtgaccctgaagaagttccccctggacaccctgatccctgatggcaaaagaatcatctgggactctaggaaaggctttatcatctccaatgccacatacaaagagattggcctgctgacctgtgaggctactgtcaatggccacctgtacaaaacaaattacctgacccacagacagaccaacacaatcattgatgtggtgctgagcccatcccatggcattgagctgtctgtgggagaaaagctggtgctgaattgtacagctagaacagaacttaatgtgggcattgatttcaactgggagtaccctagctccaagcaccagcataaaaagctggtgaacagagacctgaagacccagtctggctctgagatgaaaaagttcttgagcaccctgaccattgatggagtgaccagatctgaccagggcctgtacacctgtgctgcctcctctgggctgatgacaaaaaagaacagcacctttgtgagagtgcatgagaaggataaaacccacacctgccctccttgtcctgctcctgagctgctggggggaccatctgtgttcctgttcccccccaagcccaaggataccctgatgatcagcagaaccccagaagtgacctgtgtggtggtggatgtgtcccatgaggacccagaggtgaaattcaactggtatgtggatggagtggaggtgcacaatgccaagaccaaaccaagagaggagcagtataactccacctacagggtggtgtctgtgctgactgtgctgcaccaggattggctgaatggcaaggagtacaagtgcaaggttagcaataaagctctgcctgcccccattgaaaagaccatttccaaagccaaagggcagccaagggagccccaggtgtacaccctgcccccatctagagatgagctgaccaagaaccaggtgagcctcacatgtctggtgaagggcttttacccttctgacattgctgtggagtgggaaagcaatggacagcctgagaataactataagaccacacccccagtgctggattctgatggcagttttttcctgtactctaagctgacagtggacaaatccagatggcagcagggcaatgtgttcagctgctctgtgatgcatgaggccctgcacaatcactatacacagaagagcctgagcctgagcccagggaagtga